European Patent Application EP 4 321 617 A2, published February 14, 2024. Title: CRISPR/CPF1 SYSTEMS AND METHODS. Applicant: Integrated Dna Technologies, Inc. The sequence listing filed with the application follows.

SEQUENCE LISTING (396 sequences)

SEQ ID NO: 1 - DNA, 3924 bp, synthetic construct
  source 1..3924: mol_type = other DNA
atgacccaatttgaaggttttaccaatttataccaagtttcgaagacccttcgttttgaactgattccccaaggaaaaacactcaaacatatccaggagcaagggttcattgaggaggataaagctcgcaatgaccattacaaagagttaaaaccaatcattgaccgcatctataagacttatgctgatcaatgtctccaactggtacagcttgactgggagaatctatctgcagccatagactcctatcgtaaggaaaaaaccgaagaaacacgaaatgcgctgattgaggagcaagcaacatatagaaatgcgattcatgactactttataggtcggacggataatctgacagatgccataaataagcgccatgctgaaatctataaaggactttttaaagctgaacttttcaatggaaaagttttaaagcaattagggaccgtaaccacgacagaacatgaaaatgctctactccgttcgtttgacaaatttacgacctatttttccggcttttatgaaaaccgaaaaaatgtctttagcgctgaagatatcagcacggcaattccccatcgaatcgtccaggacaatttccctaaatttaaggaaaactgccatatttttacaagattgataaccgcagttccttctttgcgggagcattttgaaaatgtcaaaaaggccattggaatctttgttagtacgtctattgaagaagtcttttcctttcccttttataatcaacttctaacccaaacgcaaattgatctttataatcaacttctcggcggcatatctagggaagcaggcacagaaaaaatcaagggacttaatgaagttctcaatctggctatccaaaaaaatgatgaaacagcccatataatcgcgtccctgccgcatcgttttattcctctttttaaacaaattctttccgatcgaaatacgttatcctttattttggaagaattcaaaagcgatgaggaagtcatccaatccttctgcaaatataaaaccctcttgagaaacgaaaatgtactggagactgcagaagcccttttcaatgaattaaattccattgatttgactcatatctttatttcccataaaaagttagaaaccatctcttcagcgctttgtgaccattgggataccttgcgcaatgcactttacgaaagacggatttctgaactcactggcaaaataacaaaaagtgccaaagaaaaagttcaaaggtcattaaaacatgaggatataaatctccaagaaattatttctgctgcaggaaaagaactatcagaagcattcaaacaaaaaacaagtgaaattctttcccatgcccatgctgcacttgaccagcctcttcccacaacattaaaaaaacaggaagaaaaagaaatcctcaaatcacagctcgattcgcttttaggcctttatcatcttcttgattggtttgctgtcgatgaaagcaatgaagtcgacccagaattctcagcacggctgacaggcattaaactagaaatggaaccaagcctttcgttttataataaagcaagaaattatgcgacaaaaaagccctattcggtggaaaaatttaaattgaattttcaaatgccaacccttgcctctggttgggatgtcaataaagaaaaaaataatggagctattttattcgtaaaaaatggtctctattaccttggtatcatgcctaaacagaaggggcgctataaagccctgtcttttgagccgacagaaaaaacatcagaaggattcgataagatgtactatgactacttcccagatgccgcaaaaatgattcctaagtgttccactcagctaaaggctgtaaccgctcattttcaaactcataccacccccattcttctctcaaataatttcattgaacctcttgaaatcacaaaagaaatttatgacctgaacaatcctgaaaaggagcctaaaaagtttcaaacggcttatgcaaagaagacaggcgatcaaaaaggctatagagaagcgctttgcaaatggattgactttacgcgggattttctctctaaatatacgaaaacaacttcaatcgatttatcttcactccgcccttcttcgcaatataaagatttaggggaatattacgccgaactgaatccgcttctctatcatatctccttccaacgaattgctgaaaaggaaatcatggatgctgtagaaacgggaaaattgtatctgttccaaatctacaataaggattttgcgaagggccatcacgggaaaccaaatctccacaccctgtattggacaggtctcttcagtcctgaaaaccttgcgaaaaccagcatcaaacttaatggtcaagcagaattgttctatcgacctaaaagccgcatgaagcggatggcccatcgtcttggggaaaaaatgctgaacaaaaaactaaaggaccagaagacaccgattccagataccctctaccaagaactgtacgattatgtcaaccaccggctaagccatgatctttccgatgaagcaagggccctgcttccaaatgttatcaccaaagaagtctcccatgaaattataaaggatcggcggtttacttccgataaatttttcttccatgttcccattacactgaattatcaagcagccaatagtcccagtaaattcaaccagcgtgtcaatgcctaccttaaggagcatccggaaacgcccatcattggtatcgatcgtggagaacgcaatctaatctatattaccgtcattgacagtactgggaaaattttggagcagcgttccctgaataccatccagcaatttgactaccaaaaaaaattggacaacagggaaaaagagcgtgttgccgcccgtcaagcctggtccgtcgtcggaacgatcaaagaccttaaacaaggctacttgtcacaggtcatccatgaaattgtagacctgatgattcattaccaagctgttgtcgtccttgaaaacctcaacttcggatttaaatcaaaacggacaggcattgccgaaaaagcagtctaccaacaatttgaaaagatgctaatagataaactcaactgtttggttctcaaagattatcctgctgagaaagtgggaggcgtcttaaacccgtatcaacttacagatcagttcacgagctttgcaaaaatgggcacgcaaagcggcttccttttctatgtaccggccccttatacctcaaagattgatcccctgactggttttgtcgatccctttgtatggaagaccattaaaaatcatgaaagtcggaagcatttcctagaaggatttgatttcctgcattatgatgtcaaaacaggtgattttatcctccattttaaaatgaatcggaatctctctttccagagagggcttcctggcttcatgccagcttgggatattgttttcgaaaagaatgaaacccaatttgatgcaaaagggacgcccttcattgcaggaaaacgaattgttcctgtaatcgaaaatcatcgttttacgggtcgttacagagacctctatcccgctaatgaactcattgcccttctggaagaaaaaggcattgtctttagagacggaagtaatatattacccaaacttttagaaaatgatgattctcatgcaattgatacgatggtcgccttgattcgcagtgtactccaaatgagaaacagcaatgccgcaacgggggaagactacatcaactctcccgttagggatctgaacggggtgtgtttcgacagtcgattccaaaatccagaatggccaatggatgcggatgccaacggagcttatcatattgccttaaaagggcagcttcttctgaaccacctcaaagaaagcaaagatctgaaattacaaaacggcatcagcaaccaagattggctggcctacattcaggaactgagaaactga

SEQ ID NO: 2 - protein, 1307 aa, synthetic construct
MTQFEGFTNLYQVSKTLRFELIPQGKTLKHIQEQGFIEEDKARNDHYKELKPIIDRIYKTYADQCLQLVQLDWENLSAAIDSYRKEKTEETRNALIEEQATYRNAIHDYFIGRTDNLTDAINKRHAEIYKGLFKAELFNGKVLKQLGTVTTTEHENALLRSFDKFTTYFSGFYENRKNVFSAEDISTAIPHRIVQDNFPKFKENCHIFTRLITAVPSLREHFENVKKAIGIFVSTSIEEVFSFPFYNQLLTQTQIDLYNQLLGGISREAGTEKIKGLNEVLNLAIQKNDETAHIIASLPHRFIPLFKQILSDRNTLSFILEEFKSDEEVIQSFCKYKTLLRNENVLETAEALFNELNSIDLTHIFISHKKLETISSALCDHWDTLRNALYERRISELTGKITKSAKEKVQRSLKHEDINLQEIISAAGKELSEAFKQKTSEILSHAHAALDQPLPTTLKKQEEKEILKSQLDSLLGLYHLLDWFAVDESNEVDPEFSARLTGIKLEMEPSLSFYNKARNYATKKPYSVEKFKLNFQMPTLASGWDVNKEKNNGAILFVKNGLYYLGIMPKQKGRYKALSFEPTEKTSEGFDKMYYDYFPDAAKMIPKCSTQLKAVTAHFQTHTTPILLSNNFIEPLEITKEIYDLNNPEKEPKKFQTAYAKKTGDQKGYREALCKWIDFTRDFLSKYTKTTSIDLSSLRPSSQYKDLGEYYAELNPLLYHISFQRIAEKEIMDAVETGKLYLFQIYNKDFAKGHHGKPNLHTLYWTGLFSPENLAKTSIKLNGQAELFYRPKSRMKRMAHRLGEKMLNKKLKDQKTPIPDTLYQELYDYVNHRLSHDLSDEARALLPNVITKEVSHEIIKDRRFTSDKFFFHVPITLNYQAANSPSKFNQRVNAYLKEHPETPIIGIDRGERNLIYITVIDSTGKILEQRSLNTIQQFDYQKKLDNREKERVAARQAWSVVGTIKDLKQGYLSQVIHEIVDLMIHYQAVVVLENLNFGFKSKRTGIAEKAVYQQFEKMLIDKLNCLVLKDYPAEKVGGVLNPYQLTDQFTSFAKMGTQSGFLFYVPAPYTSKIDPLTGFVDPFVWKTIKNHESRKHFLEGFDFLHYDVKTGDFILHFKMNRNLSFQRGLPGFMPAWDIVFEKNETQFDAKGTPFIAGKRIVPVIENHRFTGRYRDLYPANELIALLEEKGIVFRDGSNILPKLLENDDSHAIDTMVALIRSVLQMRNSNAATGEDYINSPVRDLNGVCFDSRFQNPEWPMDADANGAYHIALKGQLLLNHLKESKDLKLQNGISNQDWLAYIQELRN

SEQ ID NO: 3 - DNA, 3714 bp, synthetic construct
  source 1..3714: mol_type = other DNA
atgagcaaactggaaaaatttacgaattgttatagcctgtccaagaccctgcgtttcaaagccatccccgttggcaaaacccaggagaatattgataataaacgtctgctggttgaggatgaaaaaagagcagaagactataagggagtcaaaaaactgctggatcggtactacctgagctttataaatgacgtgctgcatagcattaaactgaaaaatctgaataactatattagtctgttccgcaagaaaacccgaacagagaaagaaaataaagagctggaaaacctggagatcaatctgcgtaaagagatcgcaaaagcttttaaaggaaatgaaggttataaaagcctgttcaaaaaagacattattgaaaccatcctgccggaatttctggatgataaagacgagatagcgctcgtgaacagcttcaacgggttcacgaccgccttcacgggctttttcgataacagggaaaatatgttttcagaggaagccaaaagcacctcgatagcgttccgttgcattaatgaaaatttgacaagatatatcagcaacatggatattttcgagaaagttgatgcgatctttgacaaacatgaagtgcaggagattaaggaaaaaattctgaacagcgattatgatgttgaggattttttcgagggggaattttttaactttgtactgacacaggaaggtatagatgtgtataatgctattatcggcgggttcgttaccgaatccggcgagaaaattaagggtctgaatgagtacatcaatctgtataaccaaaagaccaaacagaaactgccaaaattcaaaccgctgtacaagcaagtcctgagcgatcgggaaagcttgagcttttacggtgaaggttataccagcgacgaggaggtactggaggtctttcgcaataccctgaacaagaacagcgaaattttcagctccattaaaaagctggagaaactgtttaagaattttgacgagtacagcagcgcaggtatttttgtgaagaacggacctgccataagcaccattagcaaggatatttttggagagtggaatgttatccgtgataaatggaacgcggaatatgatgacatacacctgaaaaagaaggctgtggtaactgagaaatatgaagacgatcgccgcaaaagctttaaaaaaatcggcagctttagcctggagcagctgcaggaatatgcggacgccgacctgagcgtggtcgagaaactgaaggaaattattatccaaaaagtggatgagatttacaaggtatatggtagcagcgaaaaactgtttgatgcggacttcgttctggaaaaaagcctgaaaaaaaatgatgctgttgttgcgatcatgaaagacctgctcgatagcgttaagagctttgaaaattacattaaagcattctttggcgagggcaaagaaacaaacagagacgaaagcttttatggcgacttcgtcctggcttatgacatcctgttgaaggtagatcatatatatgatgcaattcgtaattacgtaacccaaaagccgtacagcaaagataagttcaaactgtatttccagaacccgcagtttatgggtggctgggacaaagacaaggagacagactatcgcgccactattctgcgttacggcagcaagtactatctcgccatcatggacaaaaaatatgcaaagtgtctgcagaaaatcgataaagacgacgtgaacggaaattacgaaaagattaattataagctgctgccagggcccaacaagatgttaccgaaagtatttttttccaaaaaatggatggcatactataacccgagcgaggatatacagaagatttacaaaaatgggaccttcaaaaagggggatatgttcaatctgaatgactgccacaaactgatcgatttttttaaagatagcatcagccgttatcctaaatggtcaaacgcgtatgattttaatttctccgaaacggagaaatataaagacattgctggtttctatcgcgaagtcgaagaacagggttataaagttagctttgaatcggccagcaagaaagaggttgataaactggtggaggagggtaagctgtatatgtttcagatttataacaaagactttagcgacaaaagccacggtactcctaatctgcatacgatgtactttaaactgctgtttgatgagaataaccacggccaaatccgtctctccggtggagcagaactttttatgcggcgtgcgagcctaaaaaaggaagaactggtggtgcatcccgccaacagcccgattgctaacaaaaatccagataatcctaagaagaccaccacactgtcgtacgatgtctataaggataaacgtttctcggaagaccagtatgaattgcatataccgatagcaattaataaatgcccaaaaaacattttcaaaatcaacactgaagttcgtgtgctgctgaaacatgatgataatccgtatgtgatcggaattgaccgtggggagagaaatctgctgtatattgtagtcgttgatggcaagggcaacatcgttgagcagtatagcctgaatgaaataattaataattttaacggtatacgtattaaaaccgactatcatagcctgctggataaaaaggagaaagagcgttttgaggcacgccaaaattggacgagcatcgaaaacatcaaggaactgaaggcaggatatatcagccaagtagtccataaaatctgtgaactggtggagaagtacgacgctgtcattgccctggaagacctcaatagcggctttaaaaacagccgggtgaaggtggagaaacaggtataccaaaagtttgaaaagatgctcattgataagctgaactatatggttgataaaaagagcaacccgtgcgccactggcggtgcactgaaagggtaccaaattaccaataaatttgaaagctttaaaagcatgagcacgcagaatgggtttattttttatataccagcatggctgacgagcaagattgaccccagcactggttttgtcaatctgctgaaaaccaaatacacaagcattgcggatagcaaaaaatttatttcgagcttcgaccgtattatgtatgttccggaggaagatctgtttgaatttgccctggattataaaaacttcagccgcaccgatgcagattatatcaaaaaatggaagctgtacagttatggtaatcgtatacgtatcttccgtaatccgaagaaaaacaatgtgttcgattgggaagaggtctgtctgaccagcgcgtataaagaactgttcaacaagtacggaataaattatcagcaaggtgacattcgcgcactgctgtgtgaacagtcagataaagcattttatagcagctttatggcgctgatgagcctgatgctccagatgcgcaacagcataaccggtcgcacagatgttgactttctgatcagccctgtgaagaatagcgacggcatcttctacgattccaggaactatgaagcacaggaaaacgctattctgcctaaaaatgccgatgccaacggcgcctataatattgcacggaaggttctgtgggcgattggacagttcaagaaagcggaagatgagaagctggataaggtaaaaattgctattagcaataaggaatggctggagtacgcacagacatcggttaaacacgcggccgcttccctgcaggtaattaaataa

SEQ ID NO: 4 - protein, 1246 aa, synthetic construct
MLKNVGIDRLDVEKGRKNMSKLEKFTNCYSLSKTLRFKAIPVGKTQENIDNKRLLVEDEKRAEDYKGVKKLLDRYYLSFINDVLHSIKLKNLNNYISLFRKKTRTEKENKELENLEINLRKEIAKAFKGNEGYKSLFKKDIIETILPEFLDDKDEIALVNSFNGFTTAFTGFFDNRENMFSEEAKSTSIAFRCINENLTRYISNMDIFEKVDAIFDKHEVQEIKEKILNSDYDVEDFFEGEFFNFVLTQEGIDVYNAIIGGFVTESGEKIKGLNEYINLYNQKTKQKLPKFKPLYKQVLSDRESLSFYGEGYTSDEEVLEVFRNTLNKNSEIFSSIKKLEKLFKNFDEYSSAGIFVKNGPAISTISKDIFGEWNVIRDKWNAEYDDIHLKKKAVVTEKYEDDRRKSFKKIGSFSLEQLQEYADADLSVVEKLKEIIIQKVDEIYKVYGSSEKLFDADFVLEKSLKKNDAVVAIMKDLLDSVKSFENYIKAFFGEGKETNRDESFYGDFVLAYDILLKVDHIYDAIRNYVTQKPYSKDKFKLYFQNPQFMGGWDKDKETDYRATILRYGSKYYLAIMDKKYAKCLQKIDKDDVNGNYEKINYKLLPGPNKMLPKVFFSKKWMAYYNPSEDIQKIYKNGTFKKGDMFNLNDCHKLIDFFKDSISRYPKWSNAYDFNFSETEKYKDIAGFYREVEEQGYKVSFESASKKEVDKLVEEGKLYMFQIYNKDFSDKSHGTPNLHTMYFKLLFDENNHGQIRLSGGAELFMRRASLKKEELVVHPANSPIANKNPDNPKKTTTLSYDVYKDKRFSEDQYELHIPIAINKCPKNIFKINTEVRVLLKHDDNPYVIGIDRGERNLLYIVVVDGKGNIVEQYSLNEIINNFNGIRIKTDYHSLLDKKEKERFEARQNWTSIENIKELKAGYISQVVHKICELVEKYDAVIALEDLNSGFKNSRVKVEKQVYQKFEKMLIDKLNYMVDKKSNPCATGGALKGYQITNKFESFKSMSTQNGFIFYIPAWLTSKIDPSTGFVNLLKTKYTSIADSKKFISSFDRIMYVPEEDLFEFALDYKNFSRTDADYIKKWKLYSYGNRIRIFRNPKKNNVFDWEEVCLTSAYKELFNKYGINYQQGDIRALLCEQSDKAFYSSFMALMSLMLQMRNSITGRTDVDFLISPVKNSDGIFYDSRNYEAQENAILPKNADANGAYNIARKVLWAIGQFKKAEDEKLDKVKIAISNKEWLEYAQTSVKH

SEQ ID NO: 5 - DNA, 3924 bp, synthetic construct
  misc_feature 1..3924: note = Synthetic DNA
  source 1..3924: mol_type = other DNA
atgacccagtttgaaggtttcaccaatctgtatcaggttagcaaaaccctgcgttttgaactgattccgcagggtaaaaccctgaaacatattcaagaacagggcttcatcgaagaggataaagcacgtaacgatcactacaaagaactgaaaccgattatcgaccgcatctataaaacctatgcagatcagtgtctgcagctggttcagctggattgggaaaatctgagcgcagcaattgatagttatcgcaaagaaaaaaccgaagaaacccgtaatgcactgattgaagaacaggcaacctatcgtaatgccatccatgattatttcattggtcgtaccgataatctgaccgatgcaattaacaaacgtcacgccgaaatctataaaggcctgtttaaagccgaactgtttaatggcaaagttctgaaacagctgggcaccgttaccaccaccgaacatgaaaatgcactgctgcgtagctttgataaattcaccacctatttcagcggcttttatgagaatcgcaaaaacgtgtttagcgcagaagatattagcaccgcaattccgcatcgtattgtgcaggataatttcccgaaattcaaagagaactgccacatttttacccgtctgattaccgcagttccgagcctgcgtgaacattttgaaaacgttaaaaaagccatcggcatctttgttagcaccagcattgaagaagtttttagcttcccgttttacaatcagctgctgacccagacccagattgatctgtataaccaactgctgggtggtattagccgtgaagcaggcaccgaaaaaatcaaaggtctgaatgaagtgctgaatctggccattcagaaaaatgatgaaaccgcacatattattgcaagcctgccgcatcgttttattccgctgttcaaacaaattctgagcgatcgtaataccctgagctttattctggaagaattcaaatccgatgaagaggtgattcagagcttttgcaaatacaaaacgctgctgcgcaatgaaaatgttctggaaactgccgaagcactgtttaacgaactgaatagcattgatctgacccacatctttatcagccacaaaaaactggaaaccatttcaagcgcactgtgtgatcattgggataccctgcgtaatgccctgtatgaacgtcgtattagcgaactgaccggtaaaattaccaaaagcgcgaaagaaaaagttcagcgcagtctgaaacatgaggatattaatctgcaagagattattagcgcagccggtaaagaactgtcagaagcatttaaacagaaaaccagcgaaattctgtcacatgcacatgcagcactggatcagccgctgccgaccaccctgaaaaaacaagaagaaaaagaaatcctgaaaagccagctggatagcctgctgggtctgtatcatctgctggactggtttgcagttgatgaaagcaatgaagttgatccggaatttagcgcacgtctgaccggcattaaactggaaatggaaccgagcctgagcttttataacaaagcccgtaattatgccaccaaaaaaccgtatagcgtcgaaaaattcaaactgaactttcagatgccgaccctggcaagcggttgggatgttaataaagaaaaaaacaacggtgccatcctgttcgtgaaaaatggcctgtattatctgggtattatgccgaaacagaaaggtcgttataaagcgctgagctttgaaccgacggaaaaaaccagtgaaggttttgataaaatgtactacgactattttccggatgcagccaaaatgattccgaaatgtagcacccagctgaaagcagttaccgcacattttcagacccataccaccccgattctgctgagcaataactttattgaaccgctggaaatcaccaaagagatctacgatctgaataacccggaaaaagagccgaaaaaattccagaccgcatatgcaaaaaaaaccggtgatcagaaaggttatcgtgaagcgctgtgtaaatggattgatttcacccgtgattttctgagcaaatacaccaaaaccaccagtatcgatctgagcagcctgcgtccgagcagccagtataaagatctgggcgaatattatgcagaactgaatccgctgctgtatcatattagctttcagcgtattgccgagaaagaaatcatggacgcagttgaaaccggtaaactgtacctgttccagatctacaataaagattttgccaaaggccatcatggcaaaccgaatctgcataccctgtattggaccggtctgtttagccctgaaaatctggcaaaaacctcgattaaactgaatggtcaggcggaactgttttatcgtccgaaaagccgtatgaaacgtatggcacatcgtctgggtgaaaaaatgctgaacaaaaaactgaaagaccagaaaaccccgatcccggatacactgtatcaagaactgtatgattatgtgaaccatcgtctgagccatgatctgagtgatgaagcacgtgccctgctgccgaatgttattaccaaagaagttagccacgagatcattaaagatcgtcgttttaccagcgacaaattcttttttcatgtgccgattaccctgaattatcaggcagcaaatagcccgagcaaatttaaccagcgtgttaatgcatatctgaaagaacatccagaaacgccgattattggtattgatcgtggtgaacgtaacctgatttatatcaccgttattgatagcaccggcaaaatcctggaacagcgtagcctgaataccattcagcagtttgattaccagaaaaaactggataatcgcgagaaagaacgtgttgcagcacgtcaggcatggtcagttgttggtacaattaaagacctgaaacagggttatctgagccaggttattcatgaaattgtggatctgatgattcactatcaggccgttgttgtgctggaaaacctgaattttggctttaaaagcaaacgtaccggcattgcagaaaaagcagtttatcagcagttcgagaaaatgctgattgacaaactgaattgcctggtgctgaaagattatccggctgaaaaagttggtggtgttctgaatccgtatcagctgaccgatcagtttaccagctttgcaaaaatgggcacccagagcggatttctgttttatgttccggcaccgtatacgagcaaaattgatccgctgaccggttttgttgatccgtttgtttggaaaaccatcaaaaaccatgaaagccgcaaacattttctggaaggtttcgattttctgcattacgacgttaaaacgggtgatttcatcctgcactttaaaatgaatcgcaatctgagttttcagcgtggcctgcctggttttatgcctgcatgggatattgtgtttgagaaaaacgaaacacagttcgatgcaaaaggcaccccgtttattgcaggtaaacgtattgttccggtgattgaaaatcatcgtttcaccggtcgttatcgcgatctgtatccggcaaatgaactgatcgcactgctggaagagaaaggtattgtttttcgtgatggctcaaacattctgccgaaactgctggaaaatgatgatagccatgcaattgataccatggttgcactgattcgtagcgttctgcagatgcgtaatagcaatgcagcaaccggtgaagattacattaatagtccggttcgtgatctgaatggtgtttgttttgatagccgttttcagaatccggaatggccgatggatgcagatgcaaatggtgcatatcatattgcactgaaaggacagctgctgctgaaccacctgaaagaaagcaaagatctgaaactgcaaaacggcattagcaatcaggattggctggcatatatccaagaactgcgtaactga

SEQ ID NO: 6 - DNA, 3741 bp, synthetic construct
  misc_feature 1..3741: note = Synthetic DNA
  source 1..3741: mol_type = other DNA
atgctgaaaaacgtgggtattgatcgtctggatgttgaaaaaggtcgcaaaaatatgagcaaactggaaaagttcaccaactgttatagcctgagcaaaaccctgcgttttaaagcaattccggttggtaaaacccaagagaacattgataataaacgcctgctggtcgaagatgaaaaacgcgctgaagattataaaggcgtgaaaaaactgctggatcgctattatctgagcttcattaacgatgtgctgcacagcattaaactgaagaacctgaacaactatatcagcctgtttcgtaaaaaaacccgcaccgaaaaagaaaacaaagagctggaaaacctggaaatcaatctgcgtaaagaaatcgccaaagcgtttaaaggtaacgagggttataaaagcctgttcaagaaagacatcatcgaaaccattctgccggaatttctggatgataaagatgaaattgccctggtgaatagctttaatggctttaccaccgcatttaccggcttttttgataatcgcgaaaacatgttcagcgaagaagcaaaaagcaccagcattgcatttcgctgcattaatgaaaatctgacccgctacattagcaacatggatatctttgaaaaagtggacgcgatcttcgataaacacgaagtgcaagagatcaaagagaaaatcctgaacagcgattatgacgtcgaagatttttttgaaggcgagttctttaacttcgttctgacccaagaaggtatcgacgtttataacgcaattattggtggttttgttaccgaaagcggtgagaaaatcaaaggcctgaatgaatatatcaacctgtataaccagaaaaccaaacagaaactgccgaaattcaaaccgctgtataaacaggttctgagcgatcgtgaaagcctgagcttttatggtgaaggttataccagtgatgaagaggttctggaagtttttcgtaacaccctgaataaaaacagcgagatctttagcagcatcaaaaagcttgagaaactgttcaaaaactttgatgagtatagcagcgcaggcatctttgttaaaaatggtccggcaattagcaccatcagcaaagatatttttggcgaatggaatgtgatccgcgataaatggaatgccgaatatgatgatatccacctgaaaaaaaaggccgtggtgaccgagaaatatgaagatgatcgtcgtaaaagcttcaagaaaattggtagctttagcctggaacagctgcaagaatatgcagatgcagatctgagcgttgtggaaaaactgaaagaaatcatcattcagaaggtggacgagatctataaagtttatggtagcagcgaaaaactgttcgatgcagattttgttctggaaaaaagcctgaaaaagaatgatgccgttgtggccattatgaaagatctgctggatagcgttaagagcttcgagaattacatcaaagccttttttggtgagggcaaagaaaccaatcgtgatgaaagtttctatggcgattttgtgctggcctatgatattctgctgaaagtggaccatatttatgatgccattcgcaattatgttacccagaaaccgtatagcaaagacaagttcaaactgtactttcagaacccgcagtttatgggtggttgggataaagataaagaaaccgattatcgtgccaccatcctgcgttatggtagtaaatactatctggccatcatggacaaaaaatacgcaaaatgcctgcagaaaatcgacaaagatgatgtgaatggcaactatgaaaaaatcaactacaaactgctgcctggtccgaataaaatgctgccgaaagtgttctttagcaagaaatggatggcctattataacccgagcgaggatattcaaaagatctacaaaaatggcacctttaaaaagggcgacatgttcaatctgaacgattgccacaaactgatcgatttcttcaaagattcaatttcgcgttatccgaaatggtccaatgcctatgattttaactttagcgaaaccgaaaaatacaaagacattgccggtttttatcgcgaagtggaagaacagggctataaagtgagctttgaaagcgcaagcaaaaaagaggttgataagctggttgaagagggcaaactgtatatgttccagatttacaacaaagattttagcgacaaaagccatggcaccccgaatctgcataccatgtactttaaactgctgttcgacgaaaataaccatggtcagattcgtctgagcggtggtgccgaactgtttatgcgtcgtgcaagtctgaaaaaagaagaactggttgttcatccggcaaatagcccgattgcaaacaaaaatccggacaatccgaaaaaaaccacgacactgagctatgatgtgtataaagacaaacgttttagcgaggatcagtatgaactgcatatcccgattgccatcaataaatgcccgaaaaacatctttaagatcaacaccgaagttcgcgtgctgctgaaacatgatgataatccgtatgtgattggcattgatcgtggtgaacgtaacctgctgtatattgttgttgttgatggtaaaggcaacatcgtggaacagtatagtctgaacgaaattatcaacaactttaacggcatccgcatcaaaaccgactatcatagcctgctggacaagaaagaaaaagaacgttttgaagcacgtcagaactggaccagtattgaaaacatcaaagaactgaaagccggttatattagccaggtggttcataaaatctgtgagctggtagaaaaatacgatgcagttattgcactggaagatctgaatagcggtttcaaaaatagccgtgtgaaagtcgaaaaacaggtgtatcagaaattcgagaaaatgctgatcgacaaactgaactacatggtcgacaaaaaaagcaatccgtgtgcaaccggtggtgcactgaaaggttatcagattaccaacaaatttgaaagctttaaaagcatgagcacccagaacggctttatcttctatattccggcatggctgaccagcaaaattgatccgagcaccggttttgtgaacctgctgaaaacaaaatatacctccattgccgacagcaagaagtttattagcagctttgatcgcattatgtatgttccggaagaggacctgtttgaattcgcactggattacaaaaatttcagccgtaccgatgccgactacatcaaaaaatggaaactgtacagctatggtaaccgcattcgcatttttcgcaacccgaagaaaaacaatgtgttcgattgggaagaagtttgtctgaccagcgcatataaagaacttttcaacaaatacggcatcaactatcagcagggtgatattcgtgcactgctgtgtgaacagagcgataaagcgttttatagcagttttatggcactgatgagcctgatgctgcagatgcgtaatagcattaccggtcgcaccgatgtggattttctgattagtccggtgaaaaattccgatggcatcttttatgatagccgcaattacgaagcacaagaaaatgcaattctgccgaaaaacgcagatgcaaatggtgcatataacattgcacgtaaagttctgtgggcaattggccagtttaagaaagcagaagatgagaagctggacaaagtgaaaattgcgatcagcaataaagagtggctggaatacgcacagaccagcgttaaacattga

SEQ ID NO: 7 - protein, 1246 aa, synthetic construct; identical to SEQ ID NO: 4
  REGION 1..1246: note = Synthetic Amino Acid sequence

SEQ ID NO: 8 - DNA, 3924 bp, synthetic construct
  misc_feature 1..3924: note = Synthetic DNA
  source 1..3924: mol_type = other DNA
atgacccagttcgagggcttcaccaacctgtaccaggtgtccaagaccctgagattcgagctgatcccccagggcaagacactgaagcacatccaggaacagggcttcatcgaagaggacaaggcccggaacgaccactacaaagagctgaagcccatcatcgaccggatctacaagacctacgccgaccagtgcctgcagctggtgcagctggactgggagaatctgagcgccgccatcgacagctaccggaaagagaaaaccgaggaaacccggaacgccctgatcgaggaacaggccacctacagaaacgccatccacgactacttcatcggccggaccgacaacctgaccgacgccatcaacaagcggcacgccgagatctataagggcctgttcaaggccgagctgttcaacggcaaggtgctgaagcagctgggcaccgtgaccaccaccgagcacgaaaacgccctgctgcggagcttcgacaagttcaccacctacttcagcggcttctacgagaaccggaagaacgtgttcagcgccgaggacatcagcaccgccatcccccacagaatcgtgcaggacaacttccccaagttcaaagagaactgccacatcttcacccggctgatcaccgccgtgcccagcctgagagaacacttcgagaacgtgaagaaggccatcggcatcttcgtgtccaccagcatcgaggaagtgttcagcttcccattctacaaccagctgctgacccagacccagatcgacctgtataatcagctgctgggcggcatcagcagagaggccggcaccgagaagatcaagggcctgaacgaagtgctgaacctggccatccagaagaacgacgagacagcccacatcattgccagcctgccccaccggttcatccctctgttcaagcagatcctgagcgacagaaacaccctgagcttcatcctggaagagttcaagtccgatgaggaagtgatccagagcttctgcaagtataagaccctgctgaggaacgagaatgtgctggaaaccgccgaggccctgttcaatgagctgaacagcatcgacctgacccacatctttatcagccacaagaagctggaaacaatcagcagcgccctgtgcgaccactgggacacactgcggaatgccctgtacgagcggcggatctctgagctgaccggcaagatcaccaagagcgccaaagaaaaggtgcagcggagcctgaagcacgaggatatcaacctgcaggaaatcatcagcgccgctggcaaagaactgagcgaggcctttaagcagaaaaccagcgagatcctgtcccacgcccacgccgcactggatcagcctctgcctaccaccctgaagaagcaggaagagaaagagatcctgaagtcccagctggacagcctgctgggcctgtaccatctgctggattggttcgccgtggacgagagcaacgaggtggaccccgagttctccgccagactgacaggcatcaaactggaaatggaacccagcctgtccttctacaacaaggccagaaactacgccaccaagaaaccctacagcgtggaaaagtttaagctgaacttccagatgcccaccctggccagcggctgggacgtgaacaaagagaagaacaacggcgccatcctgttcgtgaagaacggactgtactacctgggcatcatgcctaagcagaagggcagatacaaggccctgtcctttgagcccaccgaaaagaccagcgagggctttgacaagatgtactacgattacttccccgacgccgccaagatgatccccaagtgcagcacccagctgaaggccgtgaccgcccactttcagacccacaccacccccatcctgctgagcaacaacttcatcgagcccctggaaatcaccaaagagatctacgacctgaacaaccccgagaaagagcccaagaagttccagaccgcctacgccaagaaaaccggcgaccagaagggctaccgcgaggctctgtgcaagtggatcgactttacccgggacttcctgagcaagtacaccaagaccacctccatcgatctgagcagcctgcggcccagctcccagtacaaggatctgggcgagtactacgccgagctgaaccctctgctgtaccacatcagcttccagcggatcgccgaaaaagaaatcatggacgccgtggaaaccggcaagctgtacctgttccagatctataacaaggacttcgccaagggccaccacggcaagcccaatctgcacaccctgtactggaccggcctgtttagccccgagaatctggccaagaccagcatcaagctgaacggccaggccgaactgttttaccggcccaagagccggatgaagcggatggcccatagactgggcgagaagatgctgaacaagaaactgaaggaccagaaaacccctatccccgacacactgtatcaggaactgtacgactacgtgaaccaccggctgagccacgacctgtccgacgaagctagagcactgctgcccaacgtgatcacaaaagaggtgtcccacgagatcatcaaggaccggcggtttacctccgataagttcttcttccacgtgcccatcaccctgaactaccaggccgccaacagccccagcaagttcaaccagagagtgaacgcctacctgaaagagcaccccgagacacccatcattggcatcgacagaggcgagcggaacctgatctacatcaccgtgatcgacagcacaggcaaaatcctggaacagagaagcctgaacaccatccagcagttcgactaccagaagaaactggacaaccgggaaaaagaacgggtggccgccagacaggcttggagcgtcgtgggcaccattaaggacctgaagcagggctacctgagccaagtgattcacgagatcgtggacctgatgatccactatcaggctgtggtggtgctggaaaacctgaacttcggcttcaagagcaagcggaccggaatcgccgagaaagccgtgtaccagcagtttgagaaaatgctgatcgacaagctgaattgcctggtgctgaaagactaccccgctgagaaagtgggaggcgtgctgaatccctaccagctgaccgaccagttcacctcctttgccaagatgggaacccagagcggcttcctgttctacgtgccagccccctacaccagcaagatcgaccctctgaccggcttcgtggaccccttcgtgtggaaaaccatcaagaaccacgagtcccggaagcacttcctggaaggctttgacttcctgcactacgacgtgaaaacaggcgatttcatcctgcacttcaagatgaatcggaatctgtccttccagaggggcctgcccggcttcatgcctgcctgggatatcgtgttcgagaagaatgagacacagttcgacgccaagggaaccccctttatcgccggcaagaggatcgtgcctgtgatcgagaaccacagattcaccggcagataccgggacctgtaccccgccaacgagctgattgccctgctggaagagaagggcatcgtgttccgggacggcagcaacatcctgcccaagctgctggaaaatgacgacagccacgccatcgataccatggtggcactgatccgcagcgtgctgcagatgcggaacagcaatgccgccaccggcgaggactacatcaatagcccagtgcgggacctgaacggcgtgtgcttcgacagcagattccagaaccccgagtggcccatggatgccgacgccaatggcgcctaccacattgccctgaagggacagctgctgctgaaccatctgaaagagagcaaagacctgaaactgcagaacggcatctccaaccaggactggctggcctatatccaggaactgcggaactga

SEQ ID NO: 9 - DNA, 683 bp, synthetic construct
  misc_feature 1..683: note = Synthetic DNA
  source 1..683: mol_type = other DNA
ccagcaagatcgatcctagcaccggattcgtgaacctgctcaagaccaagtacaccagcattgccgacagcaagaagttcatctccagcttcgaccggattatgtacgtgcccgaagaggacctgttcgaattcgccctggattacaagaacttcagccggaccgatgccgactatatcaagaagtggaagctgtatagctacggcaaccgcatccgcatcttcagaaacccgaagaaaaacaacgtgttcgactgggaagaagtgtgcctgaccagcgcctacaaagaactcttcaacaaatacggcatcaactaccagcagggcgacatcagagccctgctgtgcgagcagagcgacaaggccttttacagctccttcatggccctgatgtccctgatgctgcagatgcggaatagcatcaccggcaggaccgacgtggacttcctgatcagccctgtgaagaattccgacgggatcttctacgacagcagaaactacgaggctcaagagaacgccatcctgcctaagaacgccgatgccaacggcgcctataatatcgccagaaaggtgctgtgggccatcggccagtttaagaaggccgaggacgagaaactggacaaagtgaagatcgccatctctaacaaagagtggctggaatacgcccagaccagcgtgaaacac

SEQ ID NO: 10 - protein, 1246 aa, synthetic construct; identical to SEQ ID NO: 4
  REGION 1..1246: note = Synthetic Amino Acid Sequence

SEQ ID NO: 11 - DNA, 4086 bp, synthetic construct
  misc_feature 1..4086: note = Synthetic DNA
  source 1..4086: mol_type = other DNA
atgggtcgggatccaggtaaaccgattccgaatccgctgctgggtctggatagcaccgcaccgaaaaaaaaacgtaaagttggtattcatggtgttccggcagcaacccagtttgaaggtttcaccaatctgtatcaggttagcaaaaccctgcgttttgaactgattccgcagggtaaaaccctgaaacatattcaagaacagggcttcatcgaagaggataaagcacgtaacgatcactacaaagaactgaaaccgattatcgaccgcatctataaaacctatgcagatcagtgtctgcagctggttcagctggattgggaaaatctgagcgcagcaattgatagttatcgcaaagaaaaaaccgaagaaacccgtaatgcactgattgaagaacaggcaacctatcgtaatgccatccatgattatttcattggtcgtaccgataatctgaccgatgcaattaacaaacgtcacgccgaaatctataaaggcctgtttaaagccgaactgtttaatggcaaagttctgaaacagctgggcaccgttaccaccaccgaacatgaaaatgcactgctgcgtagctttgataaattcaccacctatttcagcggcttttatgagaatcgcaaaaacgtgtttagcgcagaagatattagcaccgcaattccgcatcgtattgtgcaggataatttcccgaaattcaaagagaactgccacatttttacccgtctgattaccgcagttccgagcctgcgtgaacattttgaaaacgttaaaaaagccatcggcatctttgttagcaccagcattgaagaagtttttagcttcccgttttacaatcagctgctgacccagacccagattgatctgtataaccaactgctgggtggtattagccgtgaagcaggcaccgaaaaaatcaaaggtctgaatgaagtgctgaatctggccattcagaaaaatgatgaaaccgcacatattattgcaagcctgccgcatcgttttattccgctgttcaaacaaattctgagcgatcgtaataccctgagctttattctggaagaattcaaatccgatgaagaggtgattcagagcttttgcaaatacaaaacgctgctgcgcaatgaaaatgttctggaaactgccgaagcactgtttaacgaactgaatagcattgatctgacccacatctttatcagccacaaaaaactggaaaccatttcaagcgcactgtgtgatcattgggataccctgcgtaatgccctgtatgaacgtcgtattagcgaactgaccggtaaaattaccaaaagcgcgaaagaaaaagttcagcgcagtctgaaacatgaggatattaatctgcaagagattattagcgcagccggtaaagaactgtcagaagcatttaaacagaaaaccagcgaaattctgtcacatgcacatgcagcactggatcagccgctgccgaccaccctgaaaaaacaagaagaaaaagaaatcctgaaaagccagctggatagcctgctgggtctgtatcatctgctggactggtttgcagttgatgaaagcaatgaagttgatccggaatttagcgcacgtctgaccggcattaaactggaaatggaaccgagcctgagcttttataacaaagcccgtaattatgccaccaaaaaaccgtatagcgtcgaaaaattcaaactgaactttcagatgccgaccctggcaagcggttgggatgttaataaagaaaaaaacaacggtgccatcctgttcgtgaaaaatggcctgtattatctgggtattatgccgaaacagaaaggtcgttataaagcgctgagctttgaaccgacggaaaaaaccagtgaaggttttgataaaatgtactacgactattttccggatgcagccaaaatgattccgaaatgtagcacccagctgaaagcagttaccgcacattttcagacccataccaccccgattctgctgagcaataactttattgaaccgctggaaatcaccaaagagatctacgatctgaataacccggaaaaagagccgaaaaaattccagaccgcatatgcaaaaaaaaccggtgatcagaaaggttatcgtgaagcgctgtgtaaatggattgatttcacccgtgattttctgagcaaatacaccaaaaccaccagtatcgatctgagcagcctgcgtccgagcagccagtataaagatctgggcgaatattatgcagaactgaatccgctgctgtatcatattagctttcagcgtattgccgagaaagaaatcatggacgcagttgaaaccggtaaactgtacctgttccagatctacaataaagattttgccaaaggccatcatggcaaaccgaatctgcataccctgtattggaccggtctgtttagccctgaaaatctggcaaaaacctcgattaaactgaatggtcaggcggaactgttttatcgtccgaaaagccgtatgaaacgtatggcacatcgtctgggtgaaaaaatgctgaacaaaaaactgaaagaccagaaaaccccgatcccggatacactgtatcaagaactgtatgattatgtgaaccatcgtctgagccatgatctgagtgatgaagcacgtgccctgctgccgaatgttattaccaaagaagttagccacgagatcattaaagatcgtcgttttaccagcgacaaattcttttttcatgtgccgattaccctgaattatcaggcagcaaatagcccgagcaaatttaaccagcgtgttaatgcatatctgaaagaacatccagaaacgccgattattggtattgatcgtggtgaacgtaacctgatttatatcaccgttattgatagcaccggcaaaatcctggaacagcgtagcctgaataccattcagcagtttgattaccagaaaaaactggataatcgcgagaaagaacgtgttgcagcacgtcaggcatggtcagttgttggtacaattaaagacctgaaacagggttatctgagccaggttattcatgaaattgtggatctgatgattcactatcaggccgttgttgtgctggaaaacctgaattttggctttaaaagcaaacgtaccggcattgcagaaaaagcagtttatcagcagttcgagaaaatgctgattgacaaactgaattgcctggtgctgaaagattatccggctgaaaaagttggtggtgttctgaatccgtatcagctgaccgatcagtttaccagctttgcaaaaatgggcacccagagcggatttctgttttatgttccggcaccgtatacgagcaaaattgatccgctgaccggttttgttgatccgtttgtttggaaaaccatcaaaaaccatgaaagccgcaaacattttctggaaggtttcgattttctgcattacgacgttaaaacgggtgatttcatcctgcactttaaaatgaatcgcaatctgagttttcagcgtggcctgcctggttttatgcctgcatgggatattgtgtttgagaaaaacgaaacacagttcgatgcaaaaggcaccccgtttattgcaggtaaacgtattgttccggtgattgaaaatcatcgtttcaccggtcgttatcgcgatctgtatccggcaaatgaactgatcgcactgctggaagagaaaggtattgtttttcgtgatggctcaaacattctgccgaaactgctggaaaatgatgatagccatgcaattgataccatggttgcactgattcgtagcgttctgcagatgcgtaatagcaatgcagcaaccggtgaagattacattaatagtccggttcgtgatctgaatggtgtttgttttgatagccgttttcagaatccggaatggccgatggatgcagatgcaaatggtgcatatcatattgcactgaaaggacagctgctgctgaaccacctgaaagaaagcaaagatctgaaactgcaaaacggcattagcaatcaggattggctggcatatatccaagaactgcgtaaccctaaaaaaaaacgcaaagtgaagcttgcggccgcactcgagcaccaccaccaccaccactga

SEQ ID NO: 12 - protein, 1361 aa, synthetic construct
  REGION 1..1361: note = Synthetic Amino Acid Sequence
MGRDPGKPIPNPLLGLDSTAPKKKRKVGIHGVPAATQFEGFTNLYQVSKTLRFELIPQGKTLKHIQEQGFIEEDKARNDHYKELKPIIDRIYKTYADQCLQLVQLDWENLSAAIDSYRKEKTEETRNALIEEQATYRNAIHDYFIGRTDNLTDAINKRHAEIYKGLFKAELFNGKVLKQLGTVTTTEHENALLRSFDKFTTYFSGFYENRKNVFSAEDISTAIPHRIVQDNFPKFKENCHIFTRLITAVPSLREHFENVKKAIGIFVSTSIEEVFSFPFYNQLLTQTQIDLYNQLLGGISREAGTEKIKGLNEVLNLAIQKNDETAHIIASLPHRFIPLFKQILSDRNTLSFILEEFKSDEEVIQSFCKYKTLLRNENVLETAEALFNELNSIDLTHIFISHKKLETISSALCDHWDTLRNALYERRISELTGKITKSAKEKVQRSLKHEDINLQEIISAAGKELSEAFKQKTSEILSHAHAALDQPLPTTLKKQEEKEILKSQLDSLLGLYHLLDWFAVDESNEVDPEFSARLTGIKLEMEPSLSFYNKARNYATKKPYSVEKFKLNFQMPTLASGWDVNKEKNNGAILFVKNGLYYLGIMPKQKGRYKALSFEPTEKTSEGFDKMYYDYFPDAAKMIPKCSTQLKAVTAHFQTHTTPILLSNNFIEPLEITKEIYDLNNPEKEPKKFQTAYAKKTGDQKGYREALCKWIDFTRDFLSKYTKTTSIDLSSLRPSSQYKDLGEYYAELNPLLYHISFQRIAEKEIMDAVETGKLYLFQIYNKDFAKGHHGKPNLHTLYWTGLFSPENLAKTSIKLNGQAELFYRPKSRMKRMAHRLGEKMLNKKLKDQKTPIPDTLYQELYDYVNHRLSHDLSDEARALLPNVITKEVSHEIIKDRRFTSDKFFFHVPITLNYQAANSPSKFNQRVNAYLKEHPETPIIGIDRGERNLIYITVIDSTGKILEQRSLNTIQQFDYQKKLDNREKERVAARQAWSVVGTIKDLKQGYLSQVIHEIVDLMIHYQAVVVLENLNFGFKSKRTGIAEKAVYQQFEKMLIDKLNCLVLKDYPAEKVGGVLNPYQLTDQFTSFAKMGTQSGFLFYVPAPYTSKIDPLTGFVDPFVWKTIKNHESRKHFLEGFDFLHYDVKTGDFILHFKMNRNLSFQRGLPGFMPAWDIVFEKNETQFDAKGTPFIAGKRIVPVIENHRFTGRYRDLYPANELIALLEEKGIVFRDGSNILPKLLENDDSHAIDTMVALIRSVLQMRNSNAATGEDYINSPVRDLNGVCFDSRFQNPEWPMDADANGAYHIALKGQLLLNHLKESKDLKLQNGISNQDWLAYIQELRNPKKKRKVKLAAALEHHHHHH

SEQ ID NO: 13 - DNA, 3876 bp, synthetic construct
  misc_feature 1..3876: note = Synthetic DNA
  source 1..3876: mol_type = other DNA
atgggtaaaccgattccgaatccgctgctgggtctggatagcaccgcaccgaaaaaaaaacgtaaagttggtattcatggtgttccggcagcactgaaaaacgtgggtattgatcgtctggatgttgaaaaaggtcgcaaaaatatgagcaaactggaaaagttcaccaactgttatagcctgagcaaaaccctgcgttttaaagcaattccggttggtaaaacccaagagaacattgataataaacgcctgctggtcgaagatgaaaaacgcgctgaagattataaaggcgtgaaaaaactgctggatcgctattatctgagcttcattaacgatgtgctgcacagcattaaactgaagaacctgaacaactatatcagcctgtttcgtaaaaaaacccgcaccgaaaaagaaaacaaagagctggaaaacctggaaatcaatctgcgtaaagaaatcgccaaagcgtttaaaggtaacgagggttataaaagcctgttcaagaaagacatcatcgaaaccattctgccggaatttctggatgataaagatgaaattgccctggtgaatagctttaatggctttaccaccgcatttaccggcttttttgataatcgcgaaaacatgttcagcgaagaagcaaaaagcaccagcattgcatttcgctgcattaatgaaaatctgacccgctacattagcaacatggatatctttgaaaaagtggacgcgatcttcgataaacacgaagtgcaagagatcaaagagaaaatcctgaacagcgattatgacgtcgaagatttttttgaaggcgagttctttaacttcgttctgacccaagaaggtatcgacgtttataacgcaattattggtggttttgttaccgaaagcggtgagaaaatcaaaggcctgaatgaatatatcaacctgtataaccagaaaaccaaacagaaactgccgaaattcaaaccgctgtataaacaggttctgagcgatcgtgaaagcctgagcttttatggtgaaggttataccagtgatgaagaggttctggaagtttttcgtaacaccctgaataaaaacagcgagatctttagcagcatcaaaaagcttgagaaactgttcaaaaactttgatgagtatagcagcgcaggcatctttgttaaaaatggtccggcaattagcaccatcagcaaagatatttttggcgaatggaatgtgatccgcgataaatggaatgccgaatatgatgatatccacctgaaaaaaaaggccgtggtgaccgagaaatatgaagatgatcgtcgtaaaagcttcaagaaaattggtagctttagcctggaacagctgcaagaatatgcagatgcagatctgagcgttgtggaaaaactgaaagaaatcatcattcagaaggtggacgagatctataaagtttatggtagcagcgaaaaactgttcgatgcagattttgttctggaaaaaagcctgaaaaagaatgatgccgttgtggccattatgaaagatctgctggatagcgttaagagcttcgagaattacatcaaagccttttttggtgagggcaaagaaaccaatcgtgatgaaagtttctatggcgattttgtgctggcctatgatattctgctgaaagtggaccatatttatgatgccattcgcaattatgttacccagaaaccgtatagcaaagacaagttcaaactgtactttcagaacccgcagtttatgggtggttgggataaagataaagaaaccgattatcgtgccaccatcctgcgttatggtagtaaatactatctggccatcatggacaaaaaatacgcaaaatgcctgcagaaaatcgacaaagatgatgtgaatggcaactatgaaaaaatcaactacaaactgctgcctggtccgaataaaatgctgccgaaagtgttctttagcaagaaatggatggcctattataacccgagcgaggatattcaaaagatctacaaaaatggcacctttaaaaagggcgacatgttcaatctgaacgattgccacaaactgatcgatttcttcaaagattcaatttcgcgttatccgaaatggtccaatgcctatgattttaactttagcgaaaccgaaaaatacaaagacattgccggtttttatcgcgaagtggaagaacagggctataaagtgagctttgaaagcgcaagcaaaaaagaggttgataagctggttgaagagggcaaactgtatatgttccagatttacaacaaagattttagcgacaaaagccatggcaccccgaatctgcataccatgtactttaaactgctgttcgacgaaaataaccatggtcagattcgtctgagcggtggtgccgaactgtttatgcgtcgtgcaagtctgaaaaaagaagaactggttgttcatccggcaaatagcccgattgcaaacaaaaatccggacaatccgaaaaaaaccacgacactgagctatgatgtgtataaagacaaacgttttagcgaggatcagtatgaactgcatatcccgattgccatcaataaatgcccgaaaaacatctttaagatcaacaccgaagttcgcgtgctgctgaaacatgatgataatccgtatgtgattggcattgatcgtggtgaacgtaacctgctgtatattgttgttgttgatggtaaaggcaacatcgtggaacagtatagtctgaacgaaattatcaacaactttaacggcatccgcatcaaaaccgactatcatagcctgctggacaagaaagaaaaagaacgttttgaagcacgtcagaactggaccagtattgaaaacatcaaagaactgaaagccggttatattagccaggtggttcataaaatctgtgagctggtagaaaaatacgatgcagttattgcactggaagatctgaatagcggtttcaaaaatagccgtgtgaaagtcgaaaaacaggtgtatcagaaattcgagaaaatgctgatcgacaaactgaactacatggtcgacaaaaaaagcaatccgtgtgcaaccggtggtgcactgaaaggttatcagattaccaacaaatttgaaagctttaaaagcatgagcacccagaacggctttatcttctatattccggcatggctgaccagcaaaattgatccgagcaccggttttgtgaacctgctgaaaacaaaatatacctccattgccgacagcaagaagtttattagcagctttgatcgcattatgtatgttccggaagaggacctgtttgaattcgcactggattacaaaaatttcagccgtaccgatgccgactacatcaaaaaatggaaactgtacagctatggtaaccgcattcgcatttttcgcaacccgaagaaaaacaatgtgttcgattgggaagaagtttgtctgaccagcgcatataaagaacttttcaacaaatacggcatcaactatcagcagggtgatattcgtgcactgctgtgtgaacagagcgataaagcgttttatagcagttttatggcactgatgagcctgatgctgcagatgcgtaatagcattaccggtcgcaccgatgtggattttctgattagtccggtgaaaaattccgatggcatcttttatgatagccgcaattacgaagcacaagaaaatgcaattctgccgaaaaacgcagatgcaaatggtgcatataacattgcacgtaaagttctgtgggcaattggccagtttaagaaagcagaagatgagaagctggacaaagtgaaaattgcgatcagcaataaagagtggctggaatacgcacagaccagcgttaaacatccgaaaaaaaaacgcaaagtgctcgagcaccaccaccaccaccactga

SEQ ID NO: 14 - protein, 1291 aa, synthetic construct
  REGION 1..1291: note = Synthetic Amino Acid Sequence
MGKPIPNPLLGLDSTAPKKKRKVGIHGVPAALKNVGIDRLDVEKGRKNMSKLEKFTNCYSLSKTLRFKAIPVGKTQENIDNKRLLVEDEKRAEDYKGVKKLLDRYYLSFINDVLHSIKLKNLNNYISLFRKKTRTEKENKELENLEINLRKEIAKAFKGNEGYKSLFKKDIIETILPEFLDDKDEIALVNSFNGFTTAFTGFFDNRENMFSEEAKSTSIAFRCINENLTRYISNMDIFEKVDAIFDKHEVQEIKEKILNSDYDVEDFFEGEFFNFVLTQEGIDVYNAIIGGFVTESGEKIKGLNEYINLYNQKTKQKLPKFKPLYKQVLSDRESLSFYGEGYTSDEEVLEVFRNTLNKNSEIFSSIKKLEKLFKNFDEYSSAGIFVKNGPAISTISKDIFGEWNVIRDKWNAEYDDIHLKKKAVVTEKYEDDRRKSFKKIGSFSLEQLQEYADADLSVVEKLKEIIIQKVDEIYKVYGSSEKLFDADFVLEKSLKKNDAVVAIMKDLLDSVKSFENYIKAFFGEGKETNRDESFYGDFVLAYDILLKVDHIYDAIRNYVTQKPYSKDKFKLYFQNPQFMGGWDKDKETDYRATILRYGSKYYLAIMDKKYAKCLQKIDKDDVNGNYEKINYKLLPGPNKMLPKVFFSKKWMAYYNPSEDIQKIYKNGTFKKGDMFNLNDCHKLIDFFKDSISRYPKWSNAYDFNFSETEKYKDIAGFYREVEEQGYKVSFESASKKEVDKLVEEGKLYMFQIYNKDFSDKSHGTPNLHTMYFKLLFDENNHGQIRLSGGAELFMRRASLKKEELVVHPANSPIANKNPDNPKKTTTLSYDVYKDKRFSEDQYELHIPIAINKCPKNIFKINTEVRVLLKHDDNPYVIGIDRGERNLLYIVVVDGKGNIVEQYSLNEIINNFNGIRIKTDYHSLLDKKEKERFEARQNWTSIENIKELKAGYISQVVHKICELVEKYDAVIALEDLNSGFKNSRVKVEKQVYQKFEKMLIDKLNYMVDKKSNPCATGGALKGYQITNKFESFKSMSTQNGFIFYIPAWLTSKIDPSTGFVNLLKTKYTSIADSKKFISSFDRIMYVPEEDLFEFALDYKNFSRTDADYIKKWKLYSYGNRIRIFRNPKKNNVFDWEEVCLTSAYKELFNKYGINYQQGDIRALLCEQSDKAFYSSFMALMSLMLQMRNSITGRTDVDFLISPVKNSDGIFYDSRNYEAQENAILPKNADANGAYNIARKVLWAIGQFKKAEDEKLDKVKIAISNKEWLEYAQTSVKHPKKKRKVLEHHHHHH

SEQ ID NO: 15 - DNA, 4071 bp, synthetic construct
  misc_feature 1..4071: note = Synthetic DNA
  source 1..4071: mol_type = other DNA
atgggcaagcccattcctaatcctctgctgggcctcgacagcacagcccctaagaaaaagcggaaagtgggcatccatggcgtgccagccgccacacagtttgagggcttcaccaacctgtaccaggtgtccaagacactgcgcttcgagctgatccctcagggcaagaccctgaagcacatccaagagcagggcttcatcgaagaggacaaggcccggaacgaccactacaaagagctgaagcccatcatcgaccggatctacaagacctacgccgaccagtgtctgcagctggtgcagctcgattgggagaatctgagcgccgccatcgacagctaccggaaagagaaaaccgaggaaacccggaacgccctgatcgaggaacaggccacctacagaaacgccatccacgactacttcatcggccggaccgacaacctgaccgacgccatcaacaagagacacgccgagatctataagggcctgttcaaggccgagctgttcaacggcaaggtgctgaagcagctgggcaccgtgacaaccaccgagcacgaaaatgccctgctgcggagcttcgacaagttcaccacctacttcagcggcttctacgagaaccggaagaacgtgttcagcgccgaggacatcagcaccgccattcctcacagaatcgtgcaggacaacttccccaagttcaaagagaactgccacatcttcacccggctgatcacagccgtgcctagcctgagagaacacttcgagaacgtgaagaaggccatcggcatcttcgtgtccaccagcatcgaggaagtgttcagcttcccattctacaaccagctgctgacccagacacagatcgacctgtataatcagctgctcggcggcatcagcagagaggccggaacagagaagatcaagggcctgaacgaagtgctgaacctggccatccagaagaacgacgagacagcccacatcattgccagcctgcctcaccggttcatccctctgttcaagcagatcctgagcgacagaaacaccctgagcttcatcctggaagagttcaagtccgatgaggaagtgatccagagcttctgcaagtataagaccctgctgaggaacgagaatgtgctggaaaccgccgaggctctgtttaacgagctgaacagcatcgatctgacccacatctttatcagccacaagaagctcgagacaatcagcagcgccctgtgcgaccactgggataccctgagaaacgccctgtacgagcggagaatcagcgagctgaccggcaagatcaccaagagcgccaaagaaaaggtgcagcggagcctgaaacacgaggatatcaacctgcaagagatcatcagcgccgctggcaaagaactgagcgaggcctttaagcagaaaaccagcgagatcctgtctcacgcccacgctgctcttgatcagcctctgcctaccacactgaagaagcaagaggaaaaagagatcctgaagtcccagctggacagcctgctgggactgtaccatctgctggattggttcgccgtggacgagagcaatgaggtggaccctgagttctccgccagactgacaggcatcaagctggaaatggaacccagcctgtccttctacaacaaggccagaaactacgccaccaagaagccctacagcgtcgagaagttcaagctcaacttccagatgcctacactggccagcggctgggacgtgaacaaagagaagaacaacggcgccatcctgttcgtgaagaacggactgtactacctgggcatcatgccaaagcagaagggcagatacaaggccctgtcctttgagcccaccgaaaagaccagcgagggcttcgataagatgtactacgattacttccccgacgccgccaagatgatccccaagtgtagcacacagctgaaggccgtgaccgctcactttcagacccacaccacacctatcctgctgagcaacaacttcatcgagcccctggaaatcaccaaagagatctacgacctgaacaaccccgagaaagagcccaagaagttccagaccgcctacgccaagaaaaccggcgaccagaagggctacagagaagccctgtgcaagtggatcgactttacccgggacttcctgagcaagtacaccaagaccacctccatcgacctgagcagcctgaggcctagcagccagtataaggacctgggcgagtactacgccgagctgaatccactgctgtaccacatcagcttccagcggatcgccgaaaaagaaatcatggacgccgtggaaaccggcaagctgtacctgttccagatatacaacaaagacttcgccaagggccaccacggcaagcctaatctgcacaccctgtactggaccggcctgtttagccctgagaatctggccaagacctctatcaagctgaacggccaggccgaactgttttacagacccaagagccggatgaagcggatggcccacagactgggagagaagatgctgaacaagaaactgaaggaccagaaaacgcccattccggacacactgtaccaagagctgtacgactacgtgaaccaccggctgagccacgatctgagcgacgaagctagagcactgctgcccaacgtgatcacaaaagaggtgtcccacgagatcattaaggaccggcggtttacctccgataagttcttcttccacgtgccgatcacactgaactaccaggccgccaactctcccagcaagttcaaccagagagtgaacgcctacctgaaagagcaccccgagacacccatcattggcatcgacagaggcgagcggaacctgatctacatcaccgtgatcgactccacaggcaagatcctggaacagcggtccctgaacaccatccagcagttcgactaccagaagaagctggacaaccgagagaaagaaagagtggccgccagacaggcttggagcgttgtgggcacaatcaaggatctgaagcagggctacctgagccaagtgattcacgagatcgtggacctgatgatccactatcaggctgtggtggtgctcgagaacctgaacttcggcttcaagagcaagcggaccggaatcgccgagaaagccgtgtaccagcagtttgagaaaatgctgatcgacaagctgaattgcctggtcctgaaggactaccccgctgagaaagttggcggagtgctgaatccctaccagctgaccgatcagttcaccagctttgccaagatgggaacccagagcggcttcctgttctacgtgccagctccttacacctccaagatcgaccctctgaccggcttcgtggaccccttcgtgtggaaaaccatcaagaaccacgagtcccggaagcacttcctggaaggctttgacttcctgcactacgacgtgaaaacaggcgatttcatcctgcacttcaagatgaatcggaatctgtccttccagaggggcctgcctggcttcatgcctgcttgggatatcgtgttcgagaagaatgagactcagttcgacgccaaggggaccccttttatcgccggcaagagaattgtgcctgtgatcgagaaccacaggttcaccggcagataccgggatctgtaccccgccaatgagctgatcgccctgctggaagagaagggcatcgtgtttagagatggcagcaacatcctgcctaagctgctggaaaacgacgacagccacgccatcgataccatggtggcactgatcagatccgtgctgcagatgcggaacagcaatgccgctaccggcgaggactacatcaatagccccgtgcgggatctgaacggcgtgtgcttcgacagcagatttcagaaccccgagtggcctatggatgccgacgccaatggcgcctatcacattgccctgaaaggacagctgctgctgaaccatctgaaagagagcaaggacctgaaactgcagaacggcatctccaaccaggactggctggcctacattcaagagctgcggaatcccaaaaagaaacggaaagtgaagctggccgctgctctggaacaccaccaccatcaccat

SEQ ID NO: 16 - protein, 1357 aa, synthetic construct
  REGION 1..1357: note = Synthetic Amino Acid Sequence
MGKPIPNPLLGLDSTAPKKKRKVGIHGVPAATQFEGFTNLYQVSKTLRFELIPQGKTLKHIQEQGFIEEDKARNDHYKELKPIIDRIYKTYADQCLQLVQLDWENLSAAIDSYRKEKTEETRNALIEEQATYRNAIHDYFIGRTDNLTDAINKRHAEIYKGLFKAELFNGKVLKQLGTVTTTEHENALLRSFDKFTTYFSGFYENRKNVFSAEDISTAIPHRIVQDNFPKFKENCHIFTRLITAVPSLREHFENVKKAIGIFVSTSIEEVFSFPFYNQLLTQTQIDLYNQLLGGISREAGTEKIKGLNEVLNLAIQKNDETAHIIASLPHRFIPLFKQILSDRNTLSFILEEFKSDEEVIQSFCKYKTLLRNENVLETAEALFNELNSIDLTHIFISHKKLETISSALCDHWDTLRNALYERRISELTGKITKSAKEKVQRSLKHEDINLQEIISAAGKELSEAFKQKTSEILSHAHAALDQPLPTTLKKQEEKEILKSQLDSLLGLYHLLDWFAVDESNEVDPEFSARLTGIKLEMEPSLSFYNKARNYATKKPYSVEKFKLNFQMPTLASGWDVNKEKNNGAILFVKNGLYYLGIMPKQKGRYKALSFEPTEKTSEGFDKMYYDYFPDAAKMIPKCSTQLKAVTAHFQTHTTPILLSNNFIEPLEITKEIYDLNNPEKEPKKFQTAYAKKTGDQKGYREALCKWIDFTRDFLSKYTKTTSIDLSSLRPSSQYKDLGEYYAELNPLLYHISFQRIAEKEIMDAVETGKLYLFQIYNKDFAKGHHGKPNLHTLYWTGLFSPENLAKTSIKLNGQAELFYRPKSRMKRMAHRLGEKMLNKKLKDQKTPIPDTLYQELYDYVNHRLSHDLSDEARALLPNVITKEVSHEIIKDRRFTSDKFFFHVPITLNYQAANSPSKFNQRVNAYLKEHPETPIIGIDRGERNLIYITVIDSTGKILEQRSLNTIQQFDYQKKLDNREKERVAARQAWSVVGTIKDLKQGYLSQVIHEIVDLMIHYQAVVVLENLNFGFKSKRTGIAEKAVYQQFEKMLIDKLNCLVLKDYPAEKVGGVLNPYQLTDQFTSFAKMGTQSGFLFYVPAPYTSKIDPLTGFVDPFVWKTIKNHESRKHFLEGFDFLHYDVKTGDFILHFKMNRNLSFQRGLPGFMPAWDIVFEKNETQFDAKGTPFIAGKRIVPVIENHRFTGRYRDLYPANELIALLEEKGIVFRDGSNILPKLLENDDSHAIDTMVALIRSVLQMRNSNAATGEDYINSPVRDLNGVCFDSRFQNPEWPMDADANGAYHIALKGQLLLNHLKESKDLKLQNGISNQDWLAYIQELRNPKKKRKVKLAAALEHHHHHH

SEQ ID NO: 17 - DNA, 3873 bp, synthetic construct
  misc_feature 1..3873: note = Synthetic DNA
  source 1..3873: mol_type = other DNA
atgggcaagcccattcctaatcctctgctgggcctcgacagcacagcccctaagaaaaagcggaaagtgggcatccatggcgtgccagccgctctgaagaatgtgggcatcgacagactggacgtggaaaagggcagaaagaacatgagcaagctcgagaagttcaccaactgctacagcctgagcaagaccctgcggttcaaggccattcctgtgggcaagacccaagagaacatcgacaacaagcggctgctggtggaagatgagaagagagccgaggactacaagggcgtgaagaagctgctggaccggtactacctgagcttcatcaacgacgtgctgcacagcatcaagctgaagaacctgaacaactacatcagcctgttccggaagaaaacccggaccgagaaagagaacaaagagctggaaaacctcgagatcaacctgcggaaagagatcgccaaggccttcaagggcaacgagggctacaagagcctgttcaagaaggacatcatcgagacaatcctgcctgagttcctggacgacaaggacgagatcgccctggtcaacagcttcaacggcttcacaaccgccttcaccggctttttcgacaaccgcgagaatatgttcagcgaggaagccaagagcacctctatcgccttccggtgcatcaacgagaatctgacccggtacatcagcaacatggatatcttcgagaaggtggacgccatcttcgacaagcacgaggtgcaagagatcaaagaaaagatcctgaacagcgactacgacgtcgaggacttcttcgagggcgagttcttcaacttcgtgctgacacaagagggcatcgatgtgtacaacgccatcatcggcggcttcgtgacagagagcggcgagaagatcaagggcctgaacgagtacatcaacctctacaaccagaaaacgaagcagaagctgcccaagttcaagcccctgtacaaacaggtgctgagcgacagagagagcctgtccttttacggcgagggctataccagcgacgaagaggtgctggaagtgttcagaaacaccctgaacaagaacagcgagatcttcagctccatcaagaagctcgaaaagctgtttaagaacttcgacgagtacagcagcgccggcatcttcgtgaagaatggccctgccatcagcaccatctccaaggacatcttcggcgagtggaacgtgatccgggacaagtggaacgccgagtacgacgacatccacctgaagaaaaaggccgtggtcaccgagaagtacgaggacgacagaagaaagagcttcaagaagatcggcagcttcagcctggaacagctgcaagagtacgccgacgccgatctgagcgtggtggaaaagctgaaagagattatcatccagaaggtcgacgagatctacaaggtgtacggcagcagcgagaagctgttcgacgccgactttgtgctggaaaagagcctcaaaaagaacgacgccgtggtggccatcatgaaggacctgctggatagcgtgaagtccttcgagaactatattaaggccttctttggcgagggcaaagagacaaaccgggacgagagcttctacggcgatttcgtgctggcctacgacatcctgctgaaagtggaccacatctacgacgccatccggaactacgtgacccagaagccttacagcaaggacaagtttaagctgtacttccagaatccgcagttcatgggcggctgggacaaagacaaagaaaccgactaccgggccaccatcctgagatacggctccaagtactatctggccattatggacaagaaatacgccaagtgcctgcagaagatcgataaggacgacgtgaacggcaactacgagaagattaactacaagctgctgcccggacctaacaagatgctgcctaaggtgttctttagcaagaaatggatggcctactacaaccccagcgaggatatccagaaaatctacaagaacggcaccttcaagaaaggcgacatgttcaacctgaacgactgccacaagctgatcgatttcttcaaggacagcatcagcagataccccaagtggtccaacgcctacgacttcaatttcagcgagacagagaagtataaggatatcgccgggttctaccgcgaggtggaagaacagggctataaggtgtcctttgagagcgccagcaagaaagaggtggacaagctggtcgaagagggcaagctgtacatgttccagatctataacaaggacttctccgacaagagccacggcacccctaacctgcacaccatgtactttaagctgctgttcgatgagaacaaccacggccagatcagactgtctggcggagccgagctgtttatgagaagggccagcctgaaaaaagaggaactggtcgttcaccccgccaactctccaatcgccaacaagaaccccgacaatcccaagaaaaccaccacactgagctacgacgtgtacaaggataagcggttctccgaggaccagtacgagctgcacatccctatcgccatcaacaagtgccccaagaatatcttcaagatcaacaccgaagtgcgggtgctgctgaagcacgacgacaacccttacgtgatcggcatcgatcggggcgagagaaacctgctgtatatcgtggtggtggacggcaagggcaatatcgtggaacagtactccctgaatgagatcatcaacaacttcaatggcatccggatcaagacggactaccacagcctgctggacaaaaaagagaaagaacgcttcgaggccaggcagaactggaccagcatcgagaacatcaaagaactgaaggccggctacatctcccaggtggtgcacaagatctgcgagctggttgagaagtatgacgccgtgattgccctggaagatctgaatagcggctttaagaacagccgcgtgaaggtcgagaaacaggtgtaccagaaattcgagaagatgctgatcgacaagctgaactacatggtcgacaagaagtctaacccctgcgccacaggcggagccctgaagggatatcagatcaccaacaagttcgagtccttcaagagcatgagcacccagaatggcttcatcttctacatccccgcctggctgaccagcaagatcgatcctagcaccggattcgtgaacctgctcaagaccaagtacaccagcattgccgacagcaagaagttcatctccagcttcgaccggattatgtacgtgcccgaagaggacctgttcgaattcgccctggattacaagaacttcagccggaccgatgccgactatatcaagaagtggaagctgtatagctacggcaaccgcatccgcatcttcagaaacccgaagaaaaacaacgtgttcgactgggaagaagtgtgcctgaccagcgcctacaaagaactcttcaacaaatacggcatcaactaccagcagggcgacatcagagccctgctgtgcgagcagagcgacaaggccttttacagctccttcatggccctgatgagcctgatgctgcagatgcggaatagcatcaccggcagaaccgacgtggacttcctgatcagccccgtgaaaaactccgacggcatcttttacgacagccggaattacgaggctcaagagaacgccatcctgcctaagaacgccgatgccaacggcgcctataatatcgccagaaaggtgctgtgggccatcggccagtttaagaaggccgaggacgagaaactggacaaagtgaagatcgccatctctaacaaagagtggctggaatacgcccagaccagcgtgaagcaccccaaaaagaaacggaaagtgctggaacaccaccaccatcaccac

SEQ ID NO: 18 - DNA, 4092 bp, synthetic construct
  misc_feature 1..4092: note = Synthetic DNA
  source 1..4092: mol_type = other DNA
atgacccagtttgaaggtttcaccaatctgtatcaggttagcaaaaccctgcgttttgaactgattccgcagggtaaaaccctgaaacatattcaagaacagggcttcatcgaagaggataaagcacgtaacgatcactacaaagaactgaaaccgattatcgaccgcatctataaaacctatgcagatcagtgtctgcagctggttcagctggattgggaaaatctgagcgcagcaattgatagttatcgcaaagaaaaaaccgaagaaacccgtaatgcactgattgaagaacaggcaacctatcgtaatgccatccatgattatttcattggtcgtaccgataatctgaccgatgcaattaacaaacgtcacgccgaaatctataaaggcctgtttaaagccgaactgtttaatggcaaagttctgaaacagctgggcaccgttaccaccaccgaacatgaaaatgcactgctgcgtagctttgataaattcaccacctatttcagcggcttttatgagaatcgcaaaaacgtgtttagcgcagaagatattagcaccgcaattccgcatcgtattgtgcaggataatttcccgaaattcaaagagaactgccacatttttacccgtctgattaccgcagttccgagcctgcgtgaacattttgaaaacgttaaaaaagccatcggcatctttgttagcaccagcattgaagaagtttttagcttcccgttttacaatcagctgctgacccagacccagattgatctgtataaccaactgctgggtggtattagccgtgaagcaggcaccgaaaaaatcaaaggtctgaatgaagtgctgaatctggccattcagaaaaatgatgaaaccgcacatattattgcaagcctgccgcatcgttttattccgctgttcaaacaaattctgagcgatcgtaataccctgagctttattctggaagaattcaaatccgatgaagaggtgattcagagcttttgcaaatacaaaacgctgctgcgcaatgaaaatgttctggaaactgccgaagcactgtttaacgaactgaatagcattgatctgacccacatctttatcagccacaaaaaactggaaaccatttcaagcgcactgtgtgatcattgggataccctgcgtaatgccctgtatgaacgtcgtattagcgaactgaccggtaaaattaccaaaagcgcgaaagaaaaagttcagcgcagtctgaaacatgaggatattaatctgcaagagattattagcgcagccggtaaagaactgtcagaagcatttaaacagaaaaccagcgaaattctgtcacatgcacatgcagcactggatcagccgctgccgaccaccctgaaaaaacaagaagaaaaagaaatcctgaaaagccagctggatagcctgctgggtctgtatcatctgctggactggtttgcagttgatgaaagcaatgaagttgatccggaatttagcgcacgtctgaccggcattaaactggaaatggaaccgagcctgagcttttataacaaagcccgtaattatgccaccaaaaaaccgtatagcgtcgaaaaattcaaactgaactttcagatgccgaccctggcaagcggttgggatgttaataaagaaaaaaacaacggtgccatcctgttcgtgaaaaatggcctgtattatctgggtattatgccgaaacagaaaggtcgttataaagcgctgagctttgaaccgacggaaaaaaccagtgaaggttttgataaaatgtactacgactattttccggatgcagccaaaatgattccgaaatgtagcacccagctgaaagcagttaccgcacattttcagacccataccaccccgattctgctgagcaataactttattgaaccgctggaaatcaccaaagagatctacgatctgaataacccggaaaaagagccgaaaaaattccagaccgcatatgcaaaaaaaaccggtgatcagaaaggttatcgtgaagcgctgtgtaaatggattgatttcacccgtgattttctgagcaaatacaccaaaaccaccagtatcgatctgagcagcctgcgtccgagcagccagtataaagatctgggcgaatattatgcagaactgaatccgctgctgtatcatattagctttcagcgtattgccgagaaagaaatcatggacgcagttgaaaccggtaaactgtacctgttccagatctacaataaagattttgccaaaggccatcatggcaaaccgaatctgcataccctgtattggaccggtctgtttagccctgaaaatctggcaaaaacctcgattaaactgaatggtcaggcggaactgttttatcgtccgaaaagccgtatgaaacgtatggcacatcgtctgggtgaaaaaatgctgaacaaaaaactgaaagaccagaaaaccccgatcccggatacactgtatcaagaactgtatgattatgtgaaccatcgtctgagccatgatctgagtgatgaagcacgtgccctgctgccgaatgttattaccaaagaagttagccacgagatcattaaagatcgtcgttttaccagcgacaaattcttttttcatgtgccgattaccctgaattatcaggcagcaaatagcccgagcaaatttaaccagcgtgttaatgcatatctgaaagaacatccagaaacgccgattattggtattgatcgtggtgaacgtaacctgatttatatcaccgttattgatagcaccggcaaaatcctggaacagcgtagcctgaataccattcagcagtttgattaccagaaaaaactggataatcgcgagaaagaacgtgttgcagcacgtcaggcatggtcagttgttggtacaattaaagacctgaaacagggttatctgagccaggttattcatgaaattgtggatctgatgattcactatcaggccgttgttgtgctggaaaacctgaattttggctttaaaagcaaacgtaccggcattgcagaaaaagcagtttatcagcagttcgagaaaatgctgattgacaaactgaattgcctggtgctgaaagattatccggctgaaaaagttggtggtgttctgaatccgtatcagctgaccgatcagtttaccagctttgcaaaaatgggcacccagagcggatttctgttttatgttccggcaccgtatacgagcaaaattgatccgctgaccggttttgttgatccgtttgtttggaaaaccatcaaaaaccatgaaagccgcaaacattttctggaaggtttcgattttctgcattacgacgttaaaacgggtgatttcatcctgcactttaaaatgaatcgcaatctgagttttcagcgtggcctgcctggttttatgcctgcatgggatattgtgtttgagaaaaacgaaacacagttcgatgcaaaaggcaccccgtttattgcaggtaaacgtattgttccggtgattgaaaatcatcgtttcaccggtcgttatcgcgatctgtatccggcaaatgaactgatcgcactgctggaagagaaaggtattgtttttcgtgatggctcaaacattctgccgaaactgctggaaaatgatgatagccatgcaattgataccatggttgcactgattcgtagcgttctgcagatgcgtaatagcaatgcagcaaccggtgaagattacattaatagtccggttcgtgatctgaatggtgtttgttttgatagccgttttcagaatccggaatggccgatggatgcagatgcaaatggtgcatatcatattgcactgaaaggacagctgctgctgaaccacctgaaagaaagcaaagatctgaaactgcaaaacggcattagcaatcaggattggctggcatatatccaagaactgcgtaacggtcgtagcagtgatgatgaagcaaccgcagatagccagcatgcagcaccgcctaaaaagaaacgtaaagttggtggtagcggtggttcaggtggtagtggcggtagtggtggctcagggggttctggtggctctggtggtagcctcgagcaccaccaccaccaccactga

SEQ ID NO: 19 - protein, 1363 aa, synthetic construct
  REGION 1..1363: note = Synthetic Amino Acid Sequence
MTQFEGFTNLYQVSKTLRFELIPQGKTLKHIQEQGFIEEDKARNDHYKELKPIIDRIYKTYADQCLQLVQLDWENLSAAIDSYRKEKTEETRNALIEEQATYRNAIHDYFIGRTDNLTDAINKRHAEIYKGLFKAELFNGKVLKQLGTVTTTEHENALLRSFDKFTTYFSGFYENRKNVFSAEDISTAIPHRIVQDNFPKFKENCHIFTRLITAVPSLREHFENVKKAIGIFVSTSIEEVFSFPFYNQLLTQTQIDLYNQLLGGISREAGTEKIKGLNEVLNLAIQKNDETAHIIASLPHRFIPLFKQILSDRNTLSFILEEFKSDEEVIQSFCKYKTLLRNENVLETAEALFNELNSIDLTHIFISHKKLETISSALCDHWDTLRNALYERRISELTGKITKSAKEKVQRSLKHEDINLQEIISAAGKELSEAFKQKTSEILSHAHAALDQPLPTTLKKQEEKEILKSQLDSLLGLYHLLDWFAVDESNEVDPEFSARLTGIKLEMEPSLSFYNKARNYATKKPYSVEKFKLNFQMPTLASGWDVNKEKNNGAILFVKNGLYYLGIMPKQKGRYKALSFEPTEKTSEGFDKMYYDYFPDAAKMIPKCSTQLKAVTAHFQTHTTPILLSNNFIEPLEITKEIYDLNNPEKEPKKFQTAYAKKTGDQKGYREALCKWIDFTRDFLSKYTKTTSIDLSSLRPSSQYKDLGEYYAELNPLLYHISFQRIAEKEIMDAVETGKLYLFQIYNKDFAKGHHGKPNLHTLYWTGLFSPENLAKTSIKLNGQAELFYRPKSRMKRMAHRLGEKMLNKKLKDQKTPIPDTLYQELYDYVNHRLSHDLSDEARALLPNVITKEVSHEIIKDRRFTSDKFFFHVPITLNYQAANSPSKFNQRVNAYLKEHPETPIIGIDRGERNLIYITVIDSTGKILEQRSLNTIQQFDYQKKLDNREKERVAARQAWSVVGTIKDLKQGYLSQVIHEIVDLMIHYQAVVVLENLNFGFKSKRTGIAEKAVYQQFEKMLIDKLNCLVLKDYPAEKVGGVLNPYQLTDQFTSFAKMGTQSGFLFYVPAPYTSKIDPLTGFVDPFVWKTIKNHESRKHFLEGFDFLHYDVKTGDFILHFKMNRNLSFQRGLPGFMPAWDIVFEKNETQFDAKGTPFIAGKRIVPVIENHRFTGRYRDLYPANELIALLEEKGIVFRDGSNILPKLLENDDSHAIDTMVALIRSVLQMRNSNAATGEDYINSPVRDLNGVCFDSRFQNPEWPMDADANGAYHIALKGQLLLNHLKESKDLKLQNGISNQDWLAYIQELRNGRSSDDEATADSQHAAPPKKKRKVGGSGGSGGSGGSGGSGGSGGSGGSLEHHHHHH

SEQ ID NO: 20 - protein, 1281 aa, synthetic construct
  REGION 1..1281: note = Synthetic Amino Acid Sequence
MGDPLKNVGIDRLDVEKGRKNMSKLEKFTNCYSLSKTLRFKAIPVGKTQENIDNKRLLVEDEKRAEDYKGVKKLLDRYYLSFINDVLHSIKLKNLNNYISLFRKKTRTEKENKELENLEINLRKEIAKAFKGNEGYKSLFKKDIIETILPEFLDDKDEIALVNSFNGFTTAFTGFFDNRENMFSEEAKSTSIAFRCINENLTRYISNMDIFEKVDAIFDKHEVQEIKEKILNSDYDVEDFFEGEFFNFVLTQEGIDVYNAIIGGFVTESGEKIKGLNEYINLYNQKTKQKLPKFKPLYKQVLSDRESLSFYGEGYTSDEEVLEVFRNTLNKNSEIFSSIKKLEKLFKNFDEYSSAGIFVKNGPAISTISKDIFGEWNVIRDKWNAEYDDIHLKKKAVVTEKYEDDRRKSFKKIGSFSLEQLQEYADADLSVVEKLKEIIIQKVDEIYKVYGSSEKLFDADFVLEKSLKKNDAVVAIMKDLLDSVKSFENYIKAFFGEGKETNRDESFYGDFVLAYDILLKVDHIYDAIRNYVTQKPYSKDKFKLYFQNPQFMGGWDKDKETDYRATILRYGSKYYLAIMDKKYAKCLQKIDKDDVNGNYEKINYKLLPGPNKMLPKVFFSKKWMAYYNPSEDIQKIYKNGTFKKGDMFNLNDCHKLIDFFKDSISRYPKWSNAYDFNFSETEKYKDIAGFYREVEEQGYKVSFESASKKEVDKLVEEGKLYMFQIYNKDFSDKSHGTPNLHTMYFKLLFDENNHGQIRLSGGAELFMRRASLKKEELVVHPANSPIANKNPDNPKKTTTLSYDVYKDKRFSEDQYELHIPIAINKCPKNIFKINTEVRVLLKHDDNPYVIGIDRGERNLLYIVVVDGKGNIVEQYSLNEIINNFNGIRIKTDYHSLLDKKEKERFEARQNWTSIENIKELKAGYISQVVHKICELVEKYDAVIALEDLNSGFKNSRVKVEKQVYQKFEKMLIDKLNYMVDKKSNPCATGGALKGYQITNKFESFKSMSTQNGFIFYIPAWLTSKIDPSTGFVNLLKTKYTSIADSKKFISSFDRIMYVPEEDLFEFALDYKNFSRTDADYIKKWKLYSYGNRIRIFRNPKKNNVFDWEEVCLTSAYKELFNKYGINYQQGDIRALLCEQSDKAFYSSFMALMSLMLQMRNSITGRTDVDFLISPVKNSDGIFYDSRNYEAQENAILPKNADANGAYNIARKVLWAIGQFKKAEDEKLDKVKIAISNKEWLEYAQTSVKHGRSSDDEATADSQHAAPPKKKRKVLEHHHHHH

SEQ ID NO: 21 - DNA, 3843 bp, synthetic construct
  misc_feature 1..3843: note = Synthetic DNA
  source 1..3843: mol_type = other DNA
atgggcgaccctctgaagaacgtgggcatcgacagactggacgtggaaaagggcagaaagaacatgagcaagctcgagaagttcaccaactgctacagcctgagcaagaccctgcggttcaaggccattcctgtgggcaagacccaagagaacatcgacaacaagcggctgctggtggaagatgagaagagagccgaggactacaagggcgtgaagaagctgctggaccggtactacctgagcttcatcaacgacgtgctgcacagcatcaagctgaagaacctgaacaactacatcagcctgttccggaagaaaacccggaccgagaaagagaacaaagagctggaaaacctcgagatcaacctgcggaaagagatcgccaaggccttcaagggcaacgagggctacaagagcctgttcaagaaggacatcatcgagacaatcctgcctgagttcctggacgacaaggacgagatcgccctggtcaacagcttcaacggcttcacaaccgccttcaccggctttttcgacaaccgcgagaatatgttcagcgaggaagccaagagcacctctatcgccttccggtgcatcaacgagaatctgacccggtacatcagcaacatggatatcttcgagaaggtggacgccatcttcgacaagcacgaggtgcaagagatcaaagaaaagatcctgaacagcgactacgacgtcgaggacttcttcgagggcgagttcttcaacttcgtgctgacacaagagggcatcgatgtgtacaacgccatcatcggcggcttcgtgacagagagcggcgagaagatcaagggcctgaacgagtacatcaacctctacaaccagaaaacgaagcagaagctgcccaagttcaagcccctgtacaaacaggtgctgagcgacagagagagcctgtccttttacggcgagggctataccagcgacgaagaggtgctggaagtgttcagaaacaccctgaacaagaacagcgagatcttcagctccatcaagaagctcgaaaagctgtttaagaacttcgacgagtacagcagcgccggcatcttcgtgaagaatggccctgccatcagcaccatctccaaggacatcttcggcgagtggaacgtgatccgggacaagtggaacgccgagtacgacgacatccacctgaagaaaaaggccgtggtcaccgagaagtacgaggacgacagaagaaagagcttcaagaagatcggcagcttcagcctggaacagctgcaagagtacgccgacgccgatctgagcgtggtggaaaagctgaaagagattatcatccagaaggtcgacgagatctacaaggtgtacggcagcagcgagaagctgttcgacgccgactttgtgctggaaaagagcctcaaaaagaacgacgccgtggtggccatcatgaaggacctgctggatagcgtgaagtccttcgagaactatattaaggccttctttggcgagggcaaagagacaaaccgggacgagagcttctacggcgatttcgtgctggcctacgacatcctgctgaaagtggaccacatctacgacgccatccggaactacgtgacccagaagccttacagcaaggacaagtttaagctgtacttccagaatccgcagttcatgggcggctgggacaaagacaaagaaaccgactaccgggccaccatcctgagatacggctccaagtactatctggccattatggacaagaaatacgccaagtgcctgcagaagatcgataaggacgacgtgaacggcaactacgagaagattaactacaagctgctgcccggacctaacaagatgctgcctaaggtgttctttagcaagaaatggatggcctactacaaccccagcgaggatatccagaaaatctacaagaacggcaccttcaagaaaggcgacatgttcaacctgaacgactgccacaagctgatcgatttcttcaaggacagcatcagcagataccccaagtggtccaacgcctacgacttcaatttcagcgagacagagaagtataaggatatcgccgggttctaccgcgaggtggaagaacagggctataaggtgtcctttgagagcgccagcaagaaagaggtggacaagctggtcgaagagggcaagctgtacatgttccagatctataacaaggacttctccgacaagagccacggcacccctaacctgcacaccatgtactttaagctgctgttcgatgagaacaaccacggccagatcagactgtctggcggagccgagctgtttatgagaagggccagcctgaaaaaagaggaactggtcgttcaccccgccaactctccaatcgccaacaagaaccccgacaatcccaagaaaaccaccacactgagctacgacgtgtacaaggataagcggttctccgaggaccagtacgagctgcacatccctatcgccatcaacaagtgccccaagaatatcttcaagatcaacaccgaagtgcgggtgctgctgaagcacgacgacaacccttacgtgatcggcatcgatcggggcgagagaaacctgctgtatatcgtggtggtggacggcaagggcaatatcgtggaacagtactccctgaatgagatcatcaacaacttcaatggcatccggatcaagacggactaccacagcctgctggacaaaaaagagaaagaacgcttcgaggcccggcagaactggaccagcatcgagaacatcaaagaactgaaggccggctacatctcccaggtggtgcacaagatctgcgagctggttgagaagtatgacgccgtgattgccctggaagatctgaatagcggctttaagaacagccgcgtgaaggtcgagaaacaggtgtaccagaaattcgagaagatgctgatcgacaagctgaactacatggtcgacaagaagtctaacccctgcgccacaggcggagccctgaagggatatcagatcaccaacaagttcgagtccttcaagagcatgagcacccagaatggcttcatcttctacatccccgcctggctgaccagcaagatcgatcctagcaccggattcgtgaacctgctcaagaccaagtacaccagcattgccgacagcaagaagttcatctccagcttcgaccggattatgtacgtgcccgaagaggacctgttcgaattcgccctggattacaagaacttcagccggaccgatgccgactatatcaagaagtggaagctgtatagctacggcaaccgcatccgcatcttcagaaacccgaagaaaaacaacgtgttcgactgggaagaagtgtgcctgaccagcgcctacaaagaactcttcaacaaatacggcatcaactaccagcagggcgacatcagagccctgctgtgcgagcagagcgacaaggccttttacagctccttcatggccctgatgagcctgatgctgcagatgcggaatagcatcaccggcaggaccgacgtggacttcctgatcagccctgtgaagaattccgacgggatcttctacgacagcagaaactacgaggctcaagagaacgccatcctgcctaagaacgccgatgccaacggcgcctataatatcgccagaaaggtgctgtgggccatcggccagtttaagaaggccgaggacgagaaactggacaaagtgaagatcgccatctctaacaaagagtggctggaatacgcccagaccagcgtgaagcacggcagatctagtgacgatgaggccaccgccgatagccagcatgcagcccctccaaagaaaaagcggaaagtgctggaacaccaccaccatcaccac

SEQ ID NO: 22 - protein, 1363 aa, synthetic construct; identical to SEQ ID NO: 19
  REGION 1..1363: note = Synthetic Amino Acid Sequence

SEQ ID NO: 23 - DNA, 3846 bp, synthetic construct
  misc_feature 1..3846: note = Synthetic DNA
  source 1..3846: mol_type = other DNA
atgggggatccactgaaaaacgtgggtattgatcgtctggatgttgaaaaaggtcgcaaaaatatgagcaaactggaaaagttcaccaactgttatagcctgagcaaaaccctgcgttttaaagcaattccggttggtaaaacccaagagaacattgataataaacgcctgctggtcgaagatgaaaaacgcgctgaagattataaaggcgtgaaaaaactgctggatcgctattatctgagcttcattaacgatgtgctgcacagcattaaactgaagaacctgaacaactatatcagcctgtttcgtaaaaaaacccgcaccgaaaaagaaaacaaagagctggaaaacctggaaatcaatctgcgtaaagaaatcgccaaagcgtttaaaggtaacgagggttataaaagcctgttcaagaaagacatcatcgaaaccattctgccggaatttctggatgataaagatgaaattgccctggtgaatagctttaatggctttaccaccgcatttaccggcttttttgataatcgcgaaaacatgttcagcgaagaagcaaaaagcaccagcattgcatttcgctgcattaatgaaaatctgacccgctacattagcaacatggatatctttgaaaaagtggacgcgatcttcgataaacacgaagtgcaagagatcaaagagaaaatcctgaacagcgattatgacgtcgaagatttttttgaaggcgagttctttaacttcgttctgacccaagaaggtatcgacgtttataacgcaattattggtggttttgttaccgaaagcggtgagaaaatcaaaggcctgaatgaatatatcaacctgtataaccagaaaaccaaacagaaactgccgaaattcaaaccgctgtataaacaggttctgagcgatcgtgaaagcctgagcttttatggtgaaggttataccagtgatgaagaggttctggaagtttttcgtaacaccctgaataaaaacagcgagatctttagcagcatcaaaaagcttgagaaactgttcaaaaactttgatgagtatagcagcgcaggcatctttgttaaaaatggtccggcaattagcaccatcagcaaagatatttttggcgaatggaatgtgatccgcgataaatggaatgccgaatatgatgatatccacctgaaaaaaaaggccgtggtgaccgagaaatatgaagatgatcgtcgtaaaagcttcaagaaaattggtagctttagcctggaacagctgcaagaatatgcagatgcagatctgagcgttgtggaaaaactgaaagaaatcatcattcagaaggtggacgagatctataaagtttatggtagcagcgaaaaactgttcgatgcagattttgttctggaaaaaagcctgaaaaagaatgatgccgttgtggccattatgaaagatctgctggatagcgttaagagcttcgagaattacatcaaagccttttttggtgagggcaaagaaaccaatcgtgatgaaagtttctatggcgattttgtgctggcctatgatattctgctgaaagtggaccatatttatgatgccattcgcaattatgttacccagaaaccgtatagcaaagacaagttcaaactgtactttcagaacccgcagtttatgggtggttgggataaagataaagaaaccgattatcgtgccaccatcctgcgttatggtagtaaatactatctggccatcatggacaaaaaatacgcaaaatgcctgcagaaaatcgacaaagatgatgtgaatggcaactatgaaaaaatcaactacaaactgctgcctggtccgaataaaatgctgccgaaagtgttctttagcaagaaatggatggcctattataacccgagcgaggatattcaaaagatctacaaaaatggcacctttaaaaagggcgacatgttcaatctgaacgattgccacaaactgatcgatttcttcaaagattcaatttcgcgttatccgaaatggtccaatgcctatgattttaactttagcgaaaccgaaaaatacaaagacattgccggtttttatcgcgaagtggaagaacagggctataaagtgagctttgaaagcgcaagcaaaaaagaggttgataagctggttgaagagggcaaactgtatatgttccagatttacaacaaagattttagcgacaaaagccatggcaccccgaatctgcataccatgtactttaaactgctgttcgacgaaaataaccatggtcagattcgtctgagcggtggtgccgaactgtttatgcgtcgtgcaagtctgaaaaaagaagaactggttgttcatccggcaaatagcccgattgcaaacaaaaatccggacaatccgaaaaaaaccacgacactgagctatgatgtgtataaagacaaacgttttagcgaggatcagtatgaactgcatatcccgattgccatcaataaatgcccgaaaaacatctttaagatcaacaccgaagttcgcgtgctgctgaaacatgatgataatccgtatgtgattggcattgatcgtggtgaacgtaacctgctgtatattgttgttgttgatggtaaaggcaacatcgtggaacagtatagtctgaacgaaattatcaacaactttaacggcatccgcatcaaaaccgactatcatagcctgctggacaagaaagaaaaagaacgttttgaagcacgtcagaactggaccagtattgaaaacatcaaagaactgaaagccggttatattagccaggtggttcataaaatctgtgagctggtagaaaaatacgatgcagttattgcactggaagatctgaatagcggtttcaaaaatagccgtgtgaaagtcgaaaaacaggtgtatcagaaattcgagaaaatgctgatcgacaaactgaactacatggtcgacaaaaaaagcaatccgtgtgcaaccggtggtgcactgaaaggttatcagattaccaacaaatttgaaagctttaaaagcatgagcacccagaacggctttatcttctatattccggcatggctgaccagcaaaattgatccgagcaccggttttgtgaacctgctgaaaacaaaatatacctccattgccgacagcaagaagtttattagcagctttgatcgcattatgtatgttccggaagaggacctgtttgaattcgcactggattacaaaaatttcagccgtaccgatgccgactacatcaaaaaatggaaactgtacagctatggtaaccgcattcgcatttttcgcaacccgaagaaaaacaatgtgttcgattgggaagaagtttgtctgaccagcgcatataaagaacttttcaacaaatacggcatcaactatcagcagggtgatattcgtgcactgctgtgtgaacagagcgataaagcgttttatagcagttttatggcactgatgagcctgatgctgcagatgcgtaatagcattaccggtcgcaccgatgtggattttctgattagtccggtgaaaaattccgatggcatcttttatgatagccgcaattacgaagcacaagaaaatgcaattctgccgaaaaacgcagatgcaaatggtgcatataacattgcacgtaaagttctgtgggcaattggccagtttaagaaagcagaagatgagaagctggacaaagtgaaaattgcgatcagcaataaagagtggctggaatacgcacagaccagcgttaaacatggtcgtagcagtgatgatgaagcaaccgcagatagccagcatgcagcaccgccgaaaaaaaaacgcaaagtgctcgagcaccaccaccaccaccactga

SEQ ID NO: 24 - protein, 1278 aa, synthetic construct
  REGION 1..1278: note = Synthetic Amino Acid Sequence
MLKNVGIDRLDVEKGRKNMSKLEKFTNCYSLSKTLRFKAIPVGKTQENIDNKRLLVEDEKRAEDYKGVKKLLDRYYLSFINDVLHSIKLKNLNNYISLFRKKTRTEKENKELENLEINLRKEIAKAFKGNEGYKSLFKKDIIETILPEFLDDKDEIALVNSFNGFTTAFTGFFDNRENMFSEEAKSTSIAFRCINENLTRYISNMDIFEKVDAIFDKHEVQEIKEKILNSDYDVEDFFEGEFFNFVLTQEGIDVYNAIIGGFVTESGEKIKGLNEYINLYNQKTKQKLPKFKPLYKQVLSDRESLSFYGEGYTSDEEVLEVFRNTLNKNSEIFSSIKKLEKLFKNFDEYSSAGIFVKNGPAISTISKDIFGEWNVIRDKWNAEYDDIHLKKKAVVTEKYEDDRRKSFKKIGSFSLEQLQEYADADLSVVEKLKEIIIQKVDEIYKVYGSSEKLFDADFVLEKSLKKNDAVVAIMKDLLDSVKSFENYIKAFFGEGKETNRDESFYGDFVLAYDILLKVDHIYDAIRNYVTQKPYSKDKFKLYFQNPQFMGGWDKDKETDYRATILRYGSKYYLAIMDKKYAKCLQKIDKDDVNGNYEKINYKLLPGPNKMLPKVFFSKKWMAYYNPSEDIQKIYKNGTFKKGDMFNLNDCHKLIDFFKDSISRYPKWSNAYDFNFSETEKYKDIAGFYREVEEQGYKVSFESASKKEVDKLVEEGKLYMFQIYNKDFSDKSHGTPNLHTMYFKLLFDENNHGQIRLSGGAELFMRRASLKKEELVVHPANSPIANKNPDNPKKTTTLSYDVYKDKRFSEDQYELHIPIAINKCPKNIFKINTEVRVLLKHDDNPYVIGIDRGERNLLYIVVVDGKGNIVEQYSLNEIINNFNGIRIKTDYHSLLDKKEKERFEARQNWTSIENIKELKAGYISQVVHKICELVEKYDAVIALEDLNSGFKNSRVKVEKQVYQKFEKMLIDKLNYMVDKKSNPCATGGALKGYQITNKFESFKSMSTQNGFIFYIPAWLTSKIDPSTGFVNLLKTKYTSIADSKKFISSFDRIMYVPEEDLFEFALDYKNFSRTDADYIKKWKLYSYGNRIRIFRNPKKNNVFDWEEVCLTSAYKELFNKYGINYQQGDIRALLCEQSDKAFYSSFMALMSLMLQMRNSITGRTDVDFLISPVKNSDGIFYDSRNYEAQENAILPKNADANGAYNIARKVLWAIGQFKKAEDEKLDKVKIAISNKEWLEYAQTSVKHGRSSDDEATADSQHAAPPKKKRKVLEHHHHHH

SEQ ID NO: 25 - DNA, 21 bp, synthetic construct
  misc_feature 1..21: note = Synthetic DNA
  source 1..21: mol_type = other DNA
gtgtccaagaccctgagattc

SEQ ID NO: 26 - DNA, 20 bp, synthetic construct
  misc_feature 1..20: note = Synthetic DNA
  source 1..20: mol_type = other DNA
gggcttcagctctttgtagt

SEQ ID NO: 27 - DNA, 24 bp, synthetic construct
  misc_feature 1..24: note = Synthetic DNA
  source 1..24: mol_type = other DNA
agggcaagacactgaagcacatcc

SEQ ID NO: 28 - DNA, 20 bp, synthetic construct
  misc_feature 1..20: note = Synthetic DNA
  source 1..20: mol_type = other DNA
cagaaactacgccaccaaga

SEQ ID NO: 29 - DNA, 22 bp, synthetic construct
  misc_feature 1..22: note = Synthetic DNA
  source 1..22: mol_type = other DNA
gccgttgttcttctctttgttc

SEQ ID NO: 30 - DNA, 25 bp, synthetic construct
  misc_feature 1..25: note = Synthetic DNA
  source 1..25: mol_type = other DNA
taagctgaacttccagatgcccacc

SEQ ID NO: 31 - DNA, 22 bp, synthetic construct
  misc_feature 1..22: note = Synthetic DNA
  source 1..22: mol_type = other DNA
gtggacctgatgatccactatc

SEQ ID NO: 32 - DNA, 18 bp, synthetic construct
  misc_feature 1..18: note = Synthetic DNA
  source 1..18: mol_type = other DNA
gctggtacacggctttct

SEQ ID NO: 33 - DNA, 24 bp, synthetic construct
  misc_feature 1..24: note = Synthetic DNA
  source 1..24: mol_type = other DNA
acctgaacttcggcttcaagagca

SEQ ID NO: 34 - DNA, 22 bp, synthetic construct
  misc_feature 1..22: note = Synthetic DNA
  source 1..22: mol_type = other DNA
tgctgaaccatctgaaagagag

SEQ ID NO: 35 - DNA, 22 bp, synthetic construct
  misc_feature 1..22: note = Synthetic DNA
  source 1..22: mol_type = other DNA
gttccgcagttcctggatatag

SEQ ID NO: 36 - DNA, 23 bp, synthetic construct
  misc_feature 1..23: note = Synthetic DNA
  source 1..23: mol_type = other DNA
agtcctggttggagatgccgttc

SEQ ID NO: 37 - RNA, 44 nt, synthetic construct
  misc_feature 1..44: note = Synthetic RNA
  source 1..44: mol_type = other RNA
taatttctactcttgtagattaaacactgtttcatttcatccgt

SEQ ID NO: 38 - RNA, 44 nt, synthetic construct
  misc_feature 1..44: note = Synthetic RNA
  source 1..44: mol_type = other RNA
taatttctactcttgtagataccagcaagctgttaattacaaaa

SEQ ID NO: 39 - RNA, 44 nt, synthetic construct
  misc_feature 1..44: note = Synthetic RNA
  source 1..44: mol_type = other RNA
taatttctactcttgtagataccatctttaacctaaaagagttt

SEQ ID NO: 40 - RNA, 44 nt, synthetic construct
  misc_feature 1..44: note = Synthetic RNA
  source 1..44: mol_type = other RNA
taatttctactcttgtagatggttaaagatggttaaatgattga

SEQ ID NO: 41 - RNA, 44 nt, synthetic construct
  misc_feature 1..44: note = Synthetic RNA
  source 1..44: mol_type = other RNA
taatttctactcttgtagattgtgaaatggcttataattgctta

SEQ ID NO: 42 - RNA, 44 nt, synthetic construct
  misc_feature 1..44: note = Synthetic RNA
  source 1..44: mol_type = other RNA
taatttctactcttgtagataatgtaagtaattgcttctttttc

SEQ ID NO: 43 - RNA, 43 nt, synthetic construct
  misc_feature 1..43: note = Synthetic RNA
  source 1..43: mol_type = other RNA
aatttctactcttgtagattaaacactgtttcatttcatccgt

SEQ ID NO: 44 - RNA, 42 nt, synthetic construct
  misc_feature 1..42: note = Synthetic RNA
  source 1..42: mol_type = other RNA
atttctactcttgtagattaaacactgtttcatttcatccgt

SEQ ID NO: 45 - RNA, 41 nt, synthetic construct
  misc_feature 1..41: note = Synthetic RNA
  source 1..41: mol_type = other RNA
tttctactcttgtagattaaacactgtttcatttcatccgt

SEQ ID NO: 46 - RNA, 43 nt, synthetic construct
  misc_feature 1..43: note = Synthetic RNA
  source 1..43: mol_type = other RNA
aatttctactcttgtagataccagcaagctgttaattacaaaa

SEQ ID NO: 47 - RNA, 42 nt, synthetic construct
  misc_feature 1..42: note = Synthetic RNA
  source 1..42: mol_type = other RNA
atttctactcttgtagataccagcaagctgttaattacaaaa

SEQ ID NO: 48 - RNA, 41 nt, synthetic construct
  misc_feature 1..41: note = Synthetic RNA
  source 1..41: mol_type = other RNA
tttctactcttgtagataccagcaagctgttaattacaaaa

SEQ ID NO: 49 - RNA, 43 nt, synthetic construct
  misc_feature 1..43: note = Synthetic RNA
  source 1..43: mol_type = other RNA
aatttctactcttgtagataccatctttaacctaaaagagttt

SEQ ID NO: 50 - RNA, 42 nt, synthetic construct
  misc_feature 1..42: note = Synthetic RNA
  source 1..42: mol_type = other RNA
atttctactcttgtagataccatctttaacctaaaagagttt

SEQ ID NO: 51 - RNA, 41 nt, synthetic construct
  misc_feature 1..41: note = Synthetic RNA
  source 1..41: mol_type = other RNA
tttctactcttgtagataccatctttaacctaaaagagttt

SEQ ID NO: 52 - RNA, 43 nt, synthetic construct
  misc_feature 1..43: note = Synthetic RNA
  source 1..43: mol_type = other RNA
aatttctactcttgtagatggttaaagatggttaaatgattga

SEQ ID NO: 53 - RNA, 42 nt, synthetic construct
  misc_feature 1..42: note = Synthetic RNA
  source 1..42: mol_type = other RNA
atttctactcttgtagatggttaaagatggttaaatgattga

SEQ ID NO: 54 - RNA, 41 nt, synthetic construct
  misc_feature 1..41: note = Synthetic RNA
  source 1..41: mol_type = other RNA
tttctactcttgtagatggttaaagatggttaaatgattga

SEQ ID NO: 55 - RNA, 43 nt, synthetic construct
  misc_feature 1..43: note = Synthetic RNA
  source 1..43: mol_type = other RNA
aatttctactcttgtagattgtgaaatggcttataattgctta

SEQ ID NO: 56 - RNA, 42 nt, synthetic construct
  misc_feature 1..42: note = Synthetic RNA
  source 1..42: mol_type = other RNA
atttctactcttgtagattgtgaaatggcttataattgctta

SEQ ID NO: 57 - RNA, 41 nt, synthetic construct
  misc_feature 1..41: note = Synthetic RNA
  source 1..41: mol_type = other RNA
tttctactcttgtagattgtgaaatggcttataattgctta

SEQ ID NO: 58 - RNA, 43 nt, synthetic construct
  misc_feature 1..43: note = Synthetic RNA
  source 1..43: mol_type = other RNA
aatttctactcttgtagataatgtaagtaattgcttctttttc

SEQ ID NO: 59 - RNA, 42 nt, synthetic construct
  misc_feature 1..42: note = Synthetic RNA
  source 1..42: mol_type = other RNA
atttctactcttgtagataatgtaagtaattgcttctttttc

SEQ ID NO: 60 - RNA, 41 nt, synthetic construct
  misc_feature 1..41: note = Synthetic RNA
  source 1..41: mol_type = other RNA
tttctactcttgtagataatgtaagtaattgcttctttttc

SEQ ID NO: 61 - RNA, 41 nt, synthetic construct
  misc_feature 1..41: note = Synthetic RNA
  source 1..41: mol_type = other RNA
taatttctactcttgtagattaaacactgtttcatttcatc

SEQ ID NO: 62 - RNA, 40 nt, synthetic construct
  misc_feature 1..40: note = Synthetic RNA
  source 1..40: mol_type = other RNA
aatttctactcttgtagattaaacactgtttcatttcatc

SEQ ID NO: 63 - RNA, 39 nt, synthetic construct
  misc_feature 1..39: note = Synthetic RNA
  source 1..39: mol_type = other RNA
atttctactcttgtagattaaacactgtttcatttcatc

SEQ ID NO: 64 - RNA, 38 nt, synthetic construct
  misc_feature 1..38: note = Synthetic RNA
  source 1..38: mol_type = other RNA
tttctactcttgtagattaaacactgtttcatttcatc

SEQ ID NO: 65 - RNA, 41 nt, synthetic construct
  misc_feature 1..41: note = Synthetic RNA
  source 1..41: mol_type = other RNA
taatttctactcttgtagataccagcaagctgttaattaca

SEQ ID NO: 66 - RNA, 40 nt, synthetic construct
  misc_feature 1..40: note = Synthetic RNA
  source 1..40: mol_type = other RNA
aatttctactcttgtagataccagcaagctgttaattaca

SEQ ID NO: 67 - RNA, 39 nt, synthetic construct
  misc_feature 1..39: note = Synthetic RNA
  source 1..39: mol_type = other RNA
atttctactcttgtagataccagcaagctgttaattaca

SEQ ID NO: 68 - RNA, 38 nt, synthetic construct
  misc_feature 1..38: note = Synthetic RNA
  source 1..38: mol_type = other RNA
tttctactcttgtagataccagcaagctgttaattaca

SEQ ID NO: 69 - RNA, 41 nt, synthetic construct
  misc_feature 1..41: note = Synthetic RNA
  source 1..41: mol_type = other RNA
taatttctactcttgtagataccatctttaacctaaaagag

SEQ ID NO: 70 - RNA, 40 nt, synthetic construct
  misc_feature 1..40: note = Synthetic RNA
  source 1..40: mol_type = other RNA
aatttctactcttgtagataccatctttaacctaaaagag

SEQ ID NO: 71 - RNA, 39 nt, synthetic construct
  misc_feature 1..39: note = Synthetic RNA
  source 1..39: mol_type = other RNA
atttctactcttgtagataccatctttaacctaaaagag

SEQ ID NO: 72 - RNA, 38 nt, synthetic construct
  misc_feature 1..38: note = Synthetic RNA
  source 1..38: mol_type = other RNA
tttctactcttgtagataccatctttaacctaaaagag

SEQ ID NO: 73 - RNA, 41 nt, synthetic construct
  misc_feature 1..41: note = Synthetic RNA
  source 1..41: mol_type = other RNA
taatttctactcttgtagatggttaaagatggttaaatgat

SEQ ID NO: 74 - RNA, 40 nt, synthetic construct
  misc_feature 1..40: note = Synthetic RNA
  source 1..40: mol_type = other RNA
aatttctactcttgtagatggttaaagatggttaaatgat

SEQ ID NO: 75 - RNA, 39 nt, synthetic construct
  misc_feature 1..39: note = Synthetic RNA
  source 1..39: mol_type = other RNA
atttctactcttgtagatggttaaagatggttaaatgat

SEQ ID NO: 76 - RNA, 38 nt, synthetic construct
  misc_feature 1..38: note = Synthetic RNA
  source 1..38: mol_type = other RNA
tttctactcttgtagatggttaaagatggttaaatgat

SEQ ID NO: 77 - RNA, 41 nt, synthetic construct
  misc_feature 1..41: note = Synthetic RNA
  source 1..41: mol_type = other RNA
taatttctactcttgtagattgtgaaatggcttataattgc

SEQ ID NO: 78 - RNA, 40 nt, synthetic construct
  misc_feature 1..40: note = Synthetic RNA
  source 1..40: mol_type = other RNA
aatttctactcttgtagattgtgaaatggcttataattgc

SEQ ID NO: 79 - RNA, 39 nt, synthetic construct
  misc_feature 1..39: note = Synthetic RNA
  source 1..39: mol_type = other RNA
atttctactcttgtagattgtgaaatggcttataattgc

SEQ ID NO: 80 - RNA, 38 nt, synthetic construct
  misc_feature 1..38: note = Synthetic RNA
  source 1..38: mol_type = other RNA
tttctactcttgtagattgtgaaatggcttataattgc

SEQ ID NO: 81 - RNA, 41 nt, synthetic construct
  misc_feature 1..41: note = Synthetic RNA
  source 1..41: mol_type = other RNA
taatttctactcttgtagataatgtaagtaattgcttcttt

SEQ ID NO: 82 - RNA, 40 nt, synthetic construct
  misc_feature 1..40: note = Synthetic RNA
  source 1..40: mol_type = other RNA
aatttctactcttgtagataatgtaagtaattgcttcttt

SEQ ID NO: 83 - RNA, 39 nt, synthetic construct
  misc_feature 1..39: note = Synthetic RNA
  source 1..39: mol_type = other RNA
atttctactcttgtagataatgtaagtaattgcttcttt

SEQ ID NO: 84 - RNA, 38 nt, synthetic construct
  misc_feature 1..38: note = Synthetic RNA
  source 1..38: mol_type = other RNA
tttctactcttgtagataatgtaagtaattgcttcttt

SEQ ID NO: 85 - RNA, 39 nt, synthetic construct
  misc_feature 1..39: note = Synthetic RNA
  source 1..39: mol_type = other RNA
taatttctactcttgtagattaaacactgtttcatttca

SEQ ID NO: 86 - RNA, 38 nt, synthetic construct
  misc_feature 1..38: note = Synthetic RNA
  source 1..38: mol_type = other RNA
taatttctactcttgtagattaaacactgtttcatttc

SEQ ID NO: 87 - RNA, 37 nt, synthetic construct
  misc_feature 1..37: note = Synthetic RNA
  source 1..37: mol_type = other RNA
taatttctactcttgtagattaaacactgtttcattt

SEQ ID NO: 88 - RNA, 39 nt, synthetic construct
  misc_feature 1..39: note = Synthetic RNA
  source 1..39: mol_type = other RNA
taatttctactcttgtagataccagcaagctgttaatta

SEQ ID NO: 89 - RNA, 38 nt, synthetic construct
  misc_feature 1..38: note = Synthetic RNA
  source 1..38: mol_type = other RNA
taatttctactcttgtagataccagcaagctgttaatt

SEQ ID NO: 90 - RNA, 37 nt, synthetic construct
  misc_feature 1..37: note = Synthetic RNA
  source 1..37: mol_type = other RNA
taatttctactcttgtagataccagcaagctgttaat

SEQ ID NO: 91 - RNA, 39 nt, synthetic construct
  misc_feature 1..39: note = Synthetic RNA
  source 1..39: mol_type = other RNA
taatttctactcttgtagataccatctttaacctaaaag

SEQ ID NO: 92 - RNA, 38 nt, synthetic construct
  misc_feature 1..38: note = Synthetic RNA
  source 1..38: mol_type = other RNA
taatttctactcttgtagataccatctttaacctaaaa

SEQ ID NO: 93 - RNA, 37 nt, synthetic construct
  misc_feature 1..37: note = Synthetic RNA
  source 1..37: mol_type = other RNA
taatttctactcttgtagataccatctttaacctaaa

SEQ ID NO: 94 - RNA, 39 nt, synthetic construct
  misc_feature 1..39: note = Synthetic RNA
  source 1..39: mol_type = other RNA
taatttctactcttgtagatggttaaagatggttaaatg

SEQ ID NO: 95 - RNA, 38 nt, synthetic construct
  misc_feature 1..38: note = Synthetic RNA
  source 1..38: mol_type = other RNA
taatttctactcttgtagatggttaaagatggttaaat

SEQ ID NO: 96 - RNA, 37 nt, synthetic construct
  misc_feature 1..37: note = Synthetic RNA
  source 1..37: mol_type = other RNA
taatttctactcttgtagatggttaaagatggttaaa

SEQ ID NO: 97 - RNA, 39 nt, synthetic construct
  misc_feature 1..39: note = Synthetic RNA
  source 1..39: mol_type = other RNA
taatttctactcttgtagattgtgaaatggcttataatt

SEQ ID NO: 98 - RNA, 38 nt, synthetic construct
  misc_feature 1..38: note = Synthetic RNA
  source 1..38: mol_type = other RNA
taatttctactcttgtagattgtgaaatggcttataat

SEQ ID NO: 99 - RNA, 37 nt, synthetic construct
  misc_feature 1..37: note = Synthetic RNA
  source 1..37: mol_type = other RNA
taatttctactcttgtagattgtgaaatggcttataa

SEQ ID NO: 100 - RNA, 39 nt, synthetic construct
  misc_feature 1..39: note = Synthetic RNA
  source 1..39: mol_type = other RNA
taatttctactcttgtagataatgtaagtaattgcttct

SEQ ID NO: 101 - RNA, 38 nt, synthetic construct
  misc_feature 1..38: note = Synthetic RNA
  source 1..38: mol_type = other RNA
taatttctactcttgtagataatgtaagtaattgcttc

SEQ ID NO: 102 - RNA, 37 nt, synthetic construct
  misc_feature 1..37: note = Synthetic RNA
  source 1..37: mol_type = other RNA
taatttctactcttgtagataatgtaagtaattgctt

SEQ ID NO: 103 - RNA, 44 nt, synthetic construct; identical to SEQ ID NO: 41
  misc_feature 1..44: note = Synthetic RNA
  source 1..44: mol_type = other RNA

SEQ ID NO: 104 - RNA, 44 nt, synthetic construct; identical to SEQ ID NO: 41
  misc_feature 1..44: note = Synthetic RNA
  source 1..44: mol_type = other RNA

SEQ ID NO: 105 - RNA, 44 nt, synthetic construct; identical to SEQ ID NO: 41
  misc_feature 1..44: note = Synthetic RNA
  source 1..44: mol_type = other RNA

SEQ ID NO: 106 - RNA, 44 nt, synthetic construct; identical to SEQ ID NO: 41
  misc_feature 1..44: note = Synthetic RNA
  source 1..44: mol_type = other RNA

SEQ ID NO: 107 - RNA, 44 nt, synthetic construct; identical to SEQ ID NO: 41
  misc_feature 1..44: note = Synthetic RNA
  source 1..44: mol_type = other RNA

SEQ ID NO: 108 - RNA, 44 nt, synthetic construct; identical to SEQ ID NO: 41
  misc_feature 1..44: note = Synthetic RNA
  source 1..44: mol_type = other RNA

SEQ ID NO: 109 - RNA, 44 nt, synthetic construct; identical to SEQ ID NO: 41
  misc_feature 1..44: note = Synthetic RNA
  source 1..44: mol_type = other RNA

SEQ ID NO: 110 - RNA, 44 nt, synthetic construct; identical to SEQ ID NO: 41
  misc_feature 1..44: note = Synthetic RNA
  source 1..44: mol_type = other RNA

SEQ ID NO: 111 - RNA, 44 nt, synthetic construct; identical to SEQ ID NO: 41
  misc_feature 1..44: note = Synthetic RNA
  source 1..44: mol_type = other RNA

SEQ ID NO: 112 - RNA, 44 nt, synthetic construct; identical to SEQ ID NO: 41
  misc_feature 1..44: note = Synthetic RNA
  source 1..44: mol_type = other RNA

SEQ ID NO: 113 - RNA, 44 nt, synthetic construct; identical to SEQ ID NO: 41
  misc_feature 1..44: note = Synthetic RNA
  source 1..44: mol_type = other RNA

SEQ ID NO: 114 - RNA, 44 nt, synthetic construct; identical to SEQ ID NO: 41
  misc_feature 1..44: note = Synthetic RNA
  source 1..44: mol_type = other RNA

SEQ ID NO: 115 - RNA, 44 nt, synthetic construct; identical to SEQ ID NO: 41
  misc_feature 1..44: note = Synthetic RNA
  source 1..44: mol_type = other RNA

SEQ ID NO: 116 - RNA, 44 nt, synthetic construct; identical to SEQ ID NO: 41
  misc_feature 1..44: note = Synthetic RNA
  source 1..44: mol_type = other RNA

SEQ ID NO: 117 - RNA, 44 nt, synthetic construct; identical to SEQ ID NO: 41
  misc_feature 1..44: note = Synthetic RNA
  source 1..44: mol_type = other RNA

SEQ ID NO: 118 - RNA, 44 nt, synthetic construct; identical to SEQ ID NO: 41
  misc_feature 1..44: note = Synthetic RNA
  source 1..44: mol_type = other RNA

SEQ ID NO: 119 - RNA, 44 nt, synthetic construct; identical to SEQ ID NO: 41
  misc_feature 1..44: note = Synthetic RNA
  source 1..44: mol_type = other RNA

SEQ ID NO: 120 - RNA, 44 nt, synthetic construct; identical to SEQ ID NO: 41
  misc_feature 1..44: note = Synthetic RNA
  source 1..44: mol_type = other RNA

SEQ ID NO: 121 - RNA, 44 nt, synthetic construct; identical to SEQ ID NO: 41
  misc_feature 1..44: note = Synthetic RNA
  source 1..44: mol_type = other RNA

SEQ ID NO: 122 - RNA, 44 nt, synthetic construct; identical to SEQ ID NO: 41
  misc_feature 1..44: note = Synthetic RNA
  source 1..44: mol_type = other RNA

SEQ ID NO: 123 - RNA, 44 nt, synthetic construct; identical to SEQ ID NO: 41
  misc_feature 1..44: note = Synthetic RNA
  source 1..44: mol_type = other RNA

SEQ ID NO: 124 - RNA, 44 nt, synthetic construct; identical to SEQ ID NO: 41
  misc_feature 1..44: note = Synthetic RNA
  source 1..44: mol_type = other RNA

SEQ ID NO: 125 - RNA, 44 nt, synthetic construct; identical to SEQ ID NO: 41
  misc_feature 1..44: note = Synthetic RNA
  source 1..44: mol_type = other RNA

SEQ ID NO: 126 - RNA, 44 nt, synthetic construct; identical to SEQ ID NO: 41
  misc_feature 1..44: note = Synthetic RNA
  source 1..44: mol_type = other RNA

SEQ ID NO: 127 - RNA, 44 nt, synthetic construct; identical to SEQ ID NO: 41
  misc_feature 1..44: note = Synthetic RNA
  source 1..44: mol_type = other RNA

SEQ ID NO: 128 - RNA, 44 nt, synthetic construct; identical to SEQ ID NO: 41
  misc_feature 1..44: note = Synthetic RNA
  source 1..44: mol_type = other RNA

SEQ ID NO: 129 - RNA, 44 nt, synthetic construct; identical to SEQ ID NO: 41
  misc_feature 1..44: note = Synthetic RNA
  source 1..44: mol_type = other RNA

SEQ ID NO: 130 - RNA, 44 nt, synthetic construct; identical to SEQ ID NO: 41
  misc_feature 1..44: note = Synthetic RNA
  source 1..44: mol_type = other RNA

SEQ ID NO: 131 - RNA, 44 nt, synthetic construct; identical to SEQ ID NO: 41
  misc_feature 1..44: note = Synthetic RNA
  source 1..44: mol_type = other RNA

SEQ ID NO: 132 - RNA, 44 nt, synthetic construct; identical to SEQ ID NO: 41
  misc_feature 1..44: note = Synthetic RNA
  source 1..44: mol_type = other RNA

SEQ ID NO: 133 - RNA, 44 nt, synthetic construct; identical to SEQ ID NO: 41
  misc_feature 1..44: note = Synthetic RNA
  source 1..44: mol_type = other RNA

SEQ ID NO: 134 - RNA, 44 nt, synthetic construct; identical to SEQ ID NO: 41
  misc_feature 1..44: note = Synthetic RNA
  source 1..44: mol_type = other RNA

SEQ ID NO: 135 - RNA, 44 nt, synthetic construct; identical to SEQ ID NO: 41
  misc_feature 1..44: note = Synthetic RNA
  source 1..44: mol_type = other RNA

SEQ ID NO: 136 - RNA, 44 nt, synthetic construct; identical to SEQ ID NO: 41
  misc_feature 1..44: note = Synthetic RNA
  source 1..44: mol_type = other RNA

SEQ ID NO: 137 - RNA, 44 nt, synthetic construct; identical to SEQ ID NO: 41
  misc_feature 1..44: note = Synthetic RNA
  source 1..44: mol_type = other RNA

SEQ ID NO: 138 - RNA, 44 nt, synthetic construct; identical to SEQ ID NO: 41
  misc_feature 1..44: note = Synthetic RNA
  source 1..44: mol_type = other RNA

SEQ ID NO: 139 - RNA, 44 nt, synthetic construct; identical to SEQ ID NO: 41
  misc_feature 1..44: note = Synthetic RNA
  source 1..44: mol_type = other RNA

SEQ ID NO: 140 - RNA, 44 nt, synthetic construct; identical to SEQ ID NO: 41
  misc_feature 1..44: note = Synthetic RNA
  source 1..44: mol_type = other RNA

SEQ ID NO: 141 - RNA, 44 nt, synthetic construct; identical to SEQ ID NO: 41
  misc_feature 1..44: note = Synthetic RNA
  source 1..44: mol_type = other RNA

SEQ ID NO: 142 - RNA, 44 nt, synthetic construct; identical to SEQ ID NO: 41
  misc_feature 1..44: note = Synthetic RNA
  source 1..44: mol_type = other RNA

SEQ ID NO: 143 - RNA, 44 nt, synthetic construct; identical to SEQ ID NO: 41
  misc_feature 1..44: note = Synthetic RNA
  source 1..44: mol_type = other RNA

SEQ ID NO: 144 - RNA, 44 nt, synthetic construct; identical to SEQ ID NO: 41
  misc_feature 1..44: note = Synthetic RNA
  source 1..44: mol_type = other RNA

SEQ ID NO: 145 - RNA, 44 nt, synthetic construct; identical to SEQ ID NO: 41
  misc_feature 1..44: note = Synthetic RNA
  source 1..44: mol_type = other RNA

SEQ ID NO: 146 - RNA, 44 nt, synthetic construct; identical to SEQ ID NO: 41
  misc_feature 1..44: note = Synthetic RNA
  source 1..44: mol_type = other RNA

SEQ ID NO: 147 - RNA, 44 nt, synthetic construct; identical to SEQ ID NO: 41
  misc_feature 1..44: note = Synthetic RNA
  source 1..44: mol_type = other RNA

SEQ ID NO: 148 - RNA, 41 nt, synthetic construct; identical to SEQ ID NO: 77
  misc_feature 1..41: note = SYNTHETIC RNA
  source 1..41: mol_type = other RNA

SEQ ID NO: 149 - RNA, 41 nt, synthetic construct; identical to SEQ ID NO: 77
  misc_feature 1..41: note = SYNTHETIC RNA
  source 1..41: mol_type = other RNA

SEQ ID NO: 150 - RNA, 41 nt, synthetic construct; identical to SEQ ID NO: 77
  misc_feature 1..41: note = SYNTHETIC RNA
  source 1..41: mol_type = other RNA

SEQ ID NO: 151 - RNA, 41 nt, synthetic construct; identical to SEQ ID NO: 77
  misc_feature 1..41: note = SYNTHETIC RNA
  source 1..41: mol_type = other RNA

SEQ ID NO: 152 - RNA, 41 nt, synthetic construct; identical to SEQ ID NO: 77
  misc_feature 1..41: note = SYNTHETIC RNA
  source 1..41: mol_type = other RNA

SEQ ID NO: 153 - RNA, 41 nt, synthetic construct; identical to SEQ ID NO: 77
  misc_feature 1..41: note = SYNTHETIC RNA
  source 1..41: mol_type = other RNA

SEQ ID NO: 154 - RNA, 41 nt, synthetic construct; identical to SEQ ID NO: 77
  misc_feature 1..41: note = SYNTHETIC RNA
  source 1..41: mol_type = other RNA

SEQ ID NO: 155 - RNA, 41 nt, synthetic construct; identical to SEQ ID NO: 77
  misc_feature 1..41: note = SYNTHETIC RNA
  source 1..41: mol_type = other RNA

SEQ ID NO: 156 - RNA, 41 nt, synthetic construct; identical to SEQ ID NO: 77
  misc_feature 1..41: note = SYNTHETIC RNA
  source 1..41: mol_type = other RNA

SEQ ID NO: 157 - RNA, 41 nt, synthetic construct; identical to SEQ ID NO: 77
  misc_feature 1..41: note = SYNTHETIC RNA
  source 1..41: mol_type = other RNA

SEQ ID NO: 158 - RNA, 41 nt, synthetic construct; identical to SEQ ID NO: 77
  misc_feature 1..41: note = SYNTHETIC RNA
  source 1..41: mol_type = other RNA

SEQ ID NO: 159 - RNA, 41 nt, synthetic construct; identical to SEQ ID NO: 77
  misc_feature 1..41: note = SYNTHETIC RNA
  source 1..41: mol_type = other RNA

SEQ ID NO: 160 - RNA, 41 nt, synthetic construct; identical to SEQ ID NO: 77
  misc_feature 1..41: note = SYNTHETIC RNA
  source 1..41: mol_type = other RNA

SEQ ID NO: 161 - RNA, 41 nt, synthetic construct; identical to SEQ ID NO: 77
  misc_feature 1..41: note = SYNTHETIC RNA
  source 1..41: mol_type = other RNA

SEQ ID NO: 162 - RNA, 41 nt, synthetic construct; identical to SEQ ID NO: 77
  misc_feature 1..41: note = SYNTHETIC RNA
  source 1..41: mol_type = other RNA

SEQ ID NO: 163 - RNA, 41 nt, synthetic construct; identical to SEQ ID NO: 77
  misc_feature 1..41: note = SYNTHETIC RNA
  source 1..41: mol_type = other RNA

SEQ ID NO: 164 - RNA, 41 nt, synthetic construct; identical to SEQ ID NO: 77
  misc_feature 1..41: note = SYNTHETIC RNA
  source 1..41: mol_type = other RNA

SEQ ID NO: 165 - RNA, 41 nt, synthetic construct; identical to SEQ ID NO: 77
  misc_feature 1..41: note = SYNTHETIC RNA
  source 1..41: mol_type = other RNA

SEQ ID NO: 166 - RNA, 41 nt, synthetic construct; identical to SEQ ID NO: 77
  misc_feature 1..41: note = SYNTHETIC RNA
  source 1..41: mol_type = other RNA

SEQ ID NO: 167 - RNA, 41 nt, synthetic construct; identical to SEQ ID NO: 77
  misc_feature 1..41: note = SYNTHETIC RNA
  source 1..41: mol_type = other RNA

SEQ ID NO: 168 - RNA, 41 nt, synthetic construct; identical to SEQ ID NO: 77
  misc_feature 1..41: note = SYNTHETIC RNA
  source 1..41: mol_type = other RNA

SEQ ID NO: 169 - RNA, 41 nt, synthetic construct; identical to SEQ ID NO: 77
  misc_feature 1..41: note = SYNTHETIC RNA
  source 1..41: mol_type = other RNA

SEQ ID NO: 170 - RNA, 41 nt, synthetic construct; identical to SEQ ID NO: 77
  misc_feature 1..41: note = SYNTHETIC RNA
  source 1..41: mol_type = other RNA

SEQ ID NO: 171 - RNA, 41 nt, synthetic construct; identical to SEQ ID NO: 77
  misc_feature 1..41: note = SYNTHETIC RNA
  source 1..41: mol_type = other RNA

SEQ ID NO: 172 - RNA, 41 nt, synthetic construct; identical to SEQ ID NO: 77
  misc_feature 1..41: note = SYNTHETIC RNA
  source 1..41: mol_type = other RNA

SEQ ID NO: 173 - RNA, 41 nt, synthetic construct; identical to SEQ ID NO: 77
  misc_feature 1..41: note = SYNTHETIC RNA
  source 1..41: mol_type = other RNA

SEQ ID NO: 174 - RNA, 41 nt, synthetic construct; identical to SEQ ID NO: 77
  misc_feature 1..41: note = SYNTHETIC RNA
  source 1..41: mol_type = other RNA

SEQ ID NO: 175 - RNA, 41 nt, synthetic construct; identical to SEQ ID NO: 77
  misc_feature 1..41: note = SYNTHETIC RNA
  source 1..41: mol_type = other RNA

SEQ ID NO: 176 - RNA, 41 nt, synthetic construct; identical to SEQ ID NO: 77
  misc_feature 1..41: note = SYNTHETIC RNA
  source 1..41: mol_type = other RNA

SEQ ID NO: 177 - RNA, 41 nt, synthetic construct; identical to SEQ ID NO: 77
  misc_feature 1..41: note = SYNTHETIC RNA
  source 1..41: mol_type = other RNA

SEQ ID NO: 178 - RNA, 41 nt, synthetic construct; identical to SEQ ID NO: 77
  misc_feature 1..41: note = SYNTHETIC RNA
  source 1..41: mol_type = other RNA

SEQ ID NO: 179 - RNA, 41 nt, synthetic construct; identical to SEQ ID NO: 77
  misc_feature 1..41: note = SYNTHETIC RNA
  source 1..41: mol_type = other RNA

SEQ ID NO: 180 - RNA, 41 nt, synthetic construct; identical to SEQ ID NO: 77
  misc_feature 1..41: note = SYNTHETIC RNA
  source 1..41: mol_type = other RNA

SEQ ID NO: 181 - RNA, 41 nt, synthetic construct; identical to SEQ ID NO: 77
  misc_feature 1..41: note = SYNTHETIC RNA
  source 1..41: mol_type = other RNA

SEQ ID NO: 182 - RNA, 41 nt, synthetic construct; identical to SEQ ID NO: 77
  misc_feature 1..41: note = SYNTHETIC RNA
  source 1..41: mol_type = other RNA

SEQ ID NO: 183 - RNA, 41 nt, synthetic construct; identical to SEQ ID NO: 77
  misc_feature 1..41: note = SYNTHETIC RNA
  source 1..41: mol_type = other RNA

SEQ ID NO: 184 - RNA, 41 nt, synthetic construct; identical to SEQ ID NO: 77
  misc_feature 1..41: note = SYNTHETIC RNA
  source 1..41: mol_type = other RNA

SEQ ID NO: 185 - RNA, 41 nt, synthetic construct; identical to SEQ ID NO: 77
  misc_feature 1..41: note = SYNTHETIC RNA
  source 1..41: mol_type = other RNA

SEQ ID NO: 186 - RNA, 41 nt, synthetic construct; identical to SEQ ID NO: 77
  misc_feature 1..41: note = SYNTHETIC RNA
  source 1..41: mol_type = other RNA

SEQ ID NO: 187 - RNA, 41 nt, synthetic construct; identical to SEQ ID NO: 77
  misc_feature 1..41: note = SYNTHETIC RNA
  source 1..41: mol_type = other RNA

SEQ ID NO: 188 - RNA, 41 nt, synthetic construct; identical to SEQ ID NO: 77
  misc_feature 1..41: note = SYNTHETIC RNA
  source 1..41: mol_type = other RNA

SEQ ID NO: 189 - RNA, 44 nt, synthetic construct
  misc_feature 1..44: note = SYNTHETIC RNA
  source 1..44: mol_type = other RNA
taatttctactcttgtagatggaaagagaattgttttctccttc

SEQ ID NO: 190 - RNA, 44 nt, synthetic construct; identical to SEQ ID NO: 189
  misc_feature 1..44: note = SYNTHETIC RNA
  source 1..44: mol_type = other RNA

SEQ ID NO: 191 - RNA, 44 nt, synthetic construct; identical to SEQ ID NO: 189
  misc_feature 1..44: note = SYNTHETIC RNA
  source 1..44: mol_type = other RNA

SEQ ID NO: 192 - RNA, 44 nt, synthetic construct; identical to SEQ ID NO: 189
  misc_feature 1..44: note = SYNTHETIC RNA
  source 1..44: mol_type = other RNA

SEQ ID NO: 193 - RNA, 44 nt, synthetic construct; identical to SEQ ID NO: 189
  misc_feature 1..44: note = SYNTHETIC RNA
  source 1..44: mol_type = other RNA

SEQ ID NO: 194 - RNA, 44 nt, synthetic construct; identical to SEQ ID NO: 189
  misc_feature 1..44: note = SYNTHETIC RNA
  source 1..44: mol_type = other RNA

SEQ ID NO: 195 - RNA, 44 nt, synthetic construct; identical to SEQ ID NO: 189
  misc_feature 1..44: note = SYNTHETIC RNA
  source 1..44: mol_type = other RNA

SEQ ID NO: 196 - RNA, 44 nt, synthetic construct; identical to SEQ ID NO: 189
  misc_feature 1..44: note = SYNTHETIC RNA
  source 1..44: mol_type = other RNA

SEQ ID NO: 197 - RNA, 44 nt, synthetic construct; identical to SEQ ID NO: 189
  misc_feature 1..44: note = SYNTHETIC RNA
  source 1..44: mol_type = other RNA

SEQ ID NO: 198 - RNA, 44 nt, synthetic construct; identical to SEQ ID NO: 189
  misc_feature 1..44: note = SYNTHETIC RNA
  source 1..44: mol_type = other RNA

SEQ ID NO: 199 - RNA, 44 nt, synthetic construct; identical to SEQ ID NO: 189
  misc_feature 1..44: note = SYNTHETIC RNA
  source 1..44: mol_type = other RNA

SEQ ID NO: 200 - RNA, 44 nt, synthetic construct; identical to SEQ ID NO: 189
  misc_feature 1..44: note = SYNTHETIC RNA
  source 1..44: mol_type = other RNA

SEQ ID NO: 201 - RNA, 44 nt, synthetic construct; identical to SEQ ID NO: 189
  misc_feature 1..44: note = SYNTHETIC RNA
  source 1..44: mol_type = other RNA

SEQ ID NO: 202 - RNA, 44 nt, synthetic construct; identical to SEQ ID NO: 189
  misc_feature 1..44: note = SYNTHETIC RNA
  source 1..44: mol_type = other RNA

SEQ ID NO: 203 - RNA, 44 nt, synthetic construct; identical to SEQ ID NO: 189
  misc_feature 1..44: note = SYNTHETIC RNA
  source 1..44: mol_type = other RNA

SEQ ID NO: 204 - RNA, 44 nt, synthetic construct; identical to SEQ ID NO: 189
  misc_feature 1..44: note = SYNTHETIC RNA
  source 1..44: mol_type = other RNA

SEQ ID NO: 205 - RNA, 44 nt, synthetic construct; identical to SEQ ID NO: 189
  misc_feature 1..44: note = SYNTHETIC RNA
  source 1..44: mol_type = other RNA

SEQ ID NO: 206 - RNA, 44 nt, synthetic construct; identical to SEQ ID NO: 189
  misc_feature 1..44: note = SYNTHETIC RNA
  source 1..44: mol_type = other RNA

SEQ ID NO: 207 - RNA, 44 nt, synthetic construct; identical to SEQ ID NO: 189
  misc_feature 1..44: note = SYNTHETIC RNA
  source 1..44: mol_type = other RNA

SEQ ID NO: 208 - RNA, 44 nt, synthetic construct; identical to SEQ ID NO: 189
  misc_feature 1..44: note = SYNTHETIC RNA
  source 1..44: mol_type = other RNA

SEQ ID NO: 209 - RNA, 44 nt, synthetic construct; identical to SEQ ID NO: 189
  misc_feature 1..44: note = SYNTHETIC RNA
  source 1..44: mol_type = other RNA

SEQ ID NO: 210 - RNA, 44 nt, synthetic construct; identical to SEQ ID NO: 189
  misc_feature 1..44: note = SYNTHETIC RNA
  source 1..44: mol_type = other RNA

SEQ ID NO: 211 - RNA, 44 nt, synthetic construct; identical to SEQ ID NO: 189
  misc_feature 1..44: note = SYNTHETIC RNA
  source 1..44: mol_type = other RNA

SEQ ID NO: 212 - RNA, 44 nt, synthetic construct; identical to SEQ ID NO: 189
  misc_feature 1..44: note = SYNTHETIC RNA
  source 1..44: mol_type = other RNA

SEQ ID NO: 213 - RNA, 44 nt, synthetic construct; identical to SEQ ID NO: 189
  misc_feature 1..44: note = SYNTHETIC RNA
  source 1..44: mol_type = other RNA

SEQ ID NO: 214 - RNA, 44 nt, synthetic construct; identical to SEQ ID NO: 189
  misc_feature 1..44: note = SYNTHETIC RNA
  source 1..44: mol_type = other RNA

SEQ ID NO: 215 - RNA, 44 nt, synthetic construct; identical to SEQ ID NO: 189
  misc_feature 1..44: note = SYNTHETIC RNA
  source 1..44: mol_type = other RNA

SEQ ID NO: 216 - RNA, 44 nt, synthetic construct; identical to SEQ ID NO: 189
  misc_feature 1..44: note = SYNTHETIC RNA
  source 1..44: mol_type = other RNA

SEQ ID NO: 217 - RNA, 44 nt, synthetic construct; identical to SEQ ID NO: 189
  misc_feature 1..44: note = SYNTHETIC RNA
  source 1..44: mol_type = other RNA

SEQ ID NO: 218 - RNA, 44 nt, synthetic construct; identical to SEQ ID NO: 189
  misc_feature 1..44: note = SYNTHETIC RNA
  source 1..44: mol_type = other RNA

SEQ ID NO: 219 - RNA, 44 nt, synthetic construct; identical to SEQ ID NO: 189
  misc_feature 1..44: note = SYNTHETIC RNA
  source 1..44: mol_type = other RNA

SEQ ID NO: 220 - RNA, 44 nt, synthetic construct; identical to SEQ ID NO: 189
  misc_feature 1..44: note = SYNTHETIC RNA
  source 1..44: mol_type = other RNA

SEQ ID NO: 221 - RNA, 44 nt, synthetic construct; identical to SEQ ID NO: 189
  misc_feature 1..44: note = SYNTHETIC RNA
  source 1..44: mol_type = other RNA

SEQ ID NO: 222 - RNA, 44 nt, synthetic construct; identical to SEQ ID NO: 189
  misc_feature 1..44: note = SYNTHETIC RNA
  source 1..44: mol_type = other RNA

SEQ ID NO: 223 - RNA, 44 nt, synthetic construct; identical to SEQ ID NO: 189
  misc_feature 1..44: note = SYNTHETIC RNA
  source 1..44: mol_type = other RNA

SEQ ID NO: 224 - RNA, 44 nt, synthetic construct; identical to SEQ ID NO: 189
  misc_feature 1..44: note = SYNTHETIC RNA
  source 1..44: mol_type = other RNA

SEQ ID NO: 225 - RNA, 44 nt, synthetic construct; identical to SEQ ID NO: 189
  misc_feature 1..44: note = SYNTHETIC RNA
  source 1..44: mol_type = other RNA

SEQ ID NO: 226 - RNA, 44 nt, synthetic construct; identical to SEQ ID NO: 189
  misc_feature 1..44: note = SYNTHETIC RNA
  source 1..44: mol_type = other RNA

SEQ ID NO: 227 - RNA, 44 nt, synthetic construct; identical to SEQ ID NO: 189
  misc_feature 1..44: note = SYNTHETIC RNA
  source 1..44: mol_type = other RNA

SEQ ID NO: 228 - RNA, 44 nt, synthetic construct; identical to SEQ ID NO: 189
  misc_feature 1..44: note = SYNTHETIC RNA
  source 1..44: mol_type = other RNA

SEQ ID NO: 229 - RNA, 44 nt, synthetic construct; identical to SEQ ID NO: 189
  misc_feature 1..44: note = SYNTHETIC RNA
  source 1..44: mol_type = other RNA

SEQ ID NO: 230 - RNA, 44 nt, synthetic construct; identical to SEQ ID NO: 189
  misc_feature 1..44: note = SYNTHETIC RNA
  source 1..44: mol_type = other RNA

SEQ ID NO: 231 - RNA, 44 nt, synthetic construct; identical to SEQ ID NO: 189
  misc_feature 1..44: note = SYNTHETIC RNA
  source 1..44: mol_type = other RNA

SEQ ID NO: 232 - RNA, 44 nt, synthetic construct; identical to SEQ ID NO: 189
  misc_feature 1..44: note = SYNTHETIC RNA
  source 1..44: mol_type = other RNA

SEQ ID NO: 233 - RNA, 44 nt, synthetic construct; identical to SEQ ID NO: 189
  misc_feature 1..44: note = SYNTHETIC RNA
  source 1..44: mol_type = other RNA

SEQ ID NO: 234 - RNA, 41 nt, synthetic construct
  misc_feature 1..41: note = SYNTHETIC RNA
  source 1..41: mol_type = other RNA
taatttctactcttgtagatggaaagagaattgttttctcc

SEQ ID NO: 235 - RNA, 41 nt, synthetic construct; identical to SEQ ID NO: 234
  misc_feature 1..41: note = SYNTHETIC RNA
  source 1..41: mol_type = other RNA

SEQ ID NO: 236 - RNA, 41 nt, synthetic construct; identical to SEQ ID NO: 234
  misc_feature 1..41: note = SYNTHETIC RNA
  source 1..41: mol_type = other RNA

SEQ ID NO: 237 - RNA, 41 nt, synthetic construct; identical to SEQ ID NO: 234
  misc_feature 1..41: note = SYNTHETIC RNA
  source 1..41: mol_type = other RNA

SEQ ID NO: 238 - RNA, 41 nt, synthetic construct; identical to SEQ ID NO: 234
  misc_feature 1..41: note = SYNTHETIC RNA
  source 1..41: mol_type = other RNA

SEQ ID NO: 239 - RNA, 41 nt, synthetic construct; identical to SEQ ID NO: 234
  misc_feature 1..41: note = SYNTHETIC RNA
  source 1..41: mol_type = other RNA

SEQ ID NO: 240 - RNA, 41 nt, synthetic construct; identical to SEQ ID NO: 234
  misc_feature 1..41: note = SYNTHETIC RNA
  source 1..41: mol_type = other RNA

SEQ ID NO: 241 - RNA, 41 nt, synthetic construct; identical to SEQ ID NO: 234
  misc_feature 1..41: note = SYNTHETIC RNA
  source 1..41: mol_type = other RNA

SEQ ID NO: 242 - RNA, 41 nt, synthetic construct; identical to SEQ ID NO: 234
  misc_feature 1..41: note = SYNTHETIC RNA
  source 1..41: mol_type = other RNA

SEQ ID NO: 243 - RNA, 41 nt, synthetic construct; identical to SEQ ID NO: 234
  misc_feature 1..41: note = SYNTHETIC RNA
  source 1..41: mol_type = other RNA

SEQ ID NO: 244 - RNA, 41 nt, synthetic construct; identical to SEQ ID NO: 234
  misc_feature 1..41: note = SYNTHETIC RNA
  source 1..41: mol_type = other RNA

SEQ ID NO: 245 - RNA, 41 nt, synthetic construct; identical to SEQ ID NO: 234
  misc_feature 1..41: note = SYNTHETIC RNA
  source 1..41: mol_type = other RNA

SEQ ID NO: 246 - RNA, 41 nt, synthetic construct; identical to SEQ ID NO: 234
  misc_feature 1..41: note = SYNTHETIC RNA
  source 1..41: mol_type = other RNA

SEQ ID NO: 247 - RNA, 41 nt, synthetic construct; identical to SEQ ID NO: 234
  misc_feature 1..41: note = SYNTHETIC RNA
  source 1..41: mol_type = other RNA

SEQ ID NO: 248 - RNA, 41 nt, synthetic construct; identical to SEQ ID NO: 234
  misc_feature 1..41: note = SYNTHETIC RNA
  source 1..41: mol_type = other RNA

SEQ ID NO: 249 - RNA, 41 nt, synthetic construct; identical to SEQ ID NO: 234
  misc_feature 1..41: note = SYNTHETIC RNA
  source 1..41: mol_type = other RNA

SEQ ID NO: 250 - RNA, 41 nt, synthetic construct; identical to SEQ ID NO: 234
  misc_feature 1..41: note = SYNTHETIC RNA
  source 1..41: mol_type = other RNA

SEQ ID NO: 251 - RNA, 41 nt, synthetic construct; identical to SEQ ID NO: 234
  misc_feature 1..41: note = SYNTHETIC RNA
  source 1..41: mol_type = other RNA

SEQ ID NO: 252 - RNA, 41 nt, synthetic construct; identical to SEQ ID NO: 234
  misc_feature 1..41: note = SYNTHETIC RNA
  source 1..41: mol_type = other RNA

SEQ ID NO: 253 - RNA, 41 nt, synthetic construct; identical to SEQ ID NO: 234
  misc_feature 1..41: note = SYNTHETIC RNA
  source 1..41: mol_type = other RNA

SEQ ID NO: 254 - RNA, 41 nt, synthetic construct; identical to SEQ ID NO: 234
  misc_feature 1..41: note = SYNTHETIC RNA
  source 1..41: mol_type = other RNA

SEQ ID NO: 255 - RNA, 41 nt, synthetic construct; identical to SEQ ID NO: 234
  misc_feature 1..41: note = SYNTHETIC RNA
  source 1..41: mol_type = other RNA

SEQ ID NO: 256 - RNA, 41 nt, synthetic construct; identical to SEQ ID NO: 234
  misc_feature 1..41: note = SYNTHETIC RNA
  source 1..41: mol_type = other RNA

SEQ ID NO: 257 - RNA, 41 nt, synthetic construct; identical to SEQ ID NO: 234
  misc_feature 1..41: note = SYNTHETIC RNA
  source 1..41: mol_type = other RNA

SEQ ID NO: 258 - RNA, 41 nt, synthetic construct; identical to SEQ ID NO: 234
  misc_feature 1..41: note = SYNTHETIC RNA
  source 1..41: mol_type = other RNA

SEQ ID NO: 259 - RNA, 41 nt, synthetic construct; identical to SEQ ID NO: 234
  misc_feature 1..41: note = SYNTHETIC RNA
  source 1..41: mol_type = other RNA

SEQ ID NO: 260 - RNA, 41 nt, synthetic construct; identical to SEQ ID NO: 234
  misc_feature 1..41: note = SYNTHETIC RNA
  source 1..41: mol_type = other RNA

SEQ ID NO: 261 - RNA, 41 nt, synthetic construct; identical to SEQ ID NO: 234
  misc_feature 1..41: note = SYNTHETIC RNA
  source 1..41: mol_type = other RNA

SEQ ID NO: 262 - RNA, 41 nt, synthetic construct; identical to SEQ ID NO: 234
  misc_feature 1..41: note = SYNTHETIC RNA
  source 1..41: mol_type = other RNA

SEQ ID NO: 263 - RNA, 41 nt, synthetic construct; identical to SEQ ID NO: 234
  misc_feature 1..41: note = SYNTHETIC RNA
  source 1..41: mol_type = other RNA

SEQ ID NO: 264 - RNA, 41 nt, synthetic construct; identical to SEQ ID NO: 234
  misc_feature 1..41: note = SYNTHETIC RNA
  source 1..41: mol_type = other RNA

SEQ ID NO: 265 - RNA, 41 nt, synthetic construct; identical to SEQ ID NO: 234
  misc_feature 1..41: note = SYNTHETIC RNA
  source 1..41: mol_type = other RNA

SEQ ID NO: 266 - RNA, 41 nt, synthetic construct; identical to SEQ ID NO: 234
  misc_feature 1..41: note = SYNTHETIC RNA
  source 1..41: mol_type = other RNA

SEQ ID NO: 267 - RNA, 41 nt, synthetic construct; identical to SEQ ID NO: 234
  misc_feature 1..41: note = SYNTHETIC RNA
  source 1..41: mol_type = other RNA

SEQ ID NO: 268 - RNA, 41 nt, synthetic construct; identical to SEQ ID NO: 234
  misc_feature 1..41: note = SYNTHETIC RNA
  source 1..41: mol_type = other RNA

SEQ ID NO: 269 - RNA, 41 nt, synthetic construct; identical to SEQ ID NO: 234
  misc_feature 1..41: note = SYNTHETIC RNA
  source 1..41: mol_type = other RNA

SEQ ID NO: 270 - RNA, 41 nt, synthetic construct; identical to SEQ ID NO: 234
  misc_feature 1..41: note = SYNTHETIC RNA
  source 1..41: mol_type = other RNA

SEQ ID NO: 271 - RNA, 41 nt, synthetic construct; identical to SEQ ID NO: 234
  misc_feature 1..41: note = SYNTHETIC RNA
  source 1..41: mol_type = other RNA

SEQ ID NO: 272 - RNA, 41 nt, synthetic construct; identical to SEQ ID NO: 234
  misc_feature 1..41: note = SYNTHETIC RNA
  source 1..41: mol_type = other RNA

SEQ ID NO: 273 - RNA, 41 nt, synthetic construct; identical to SEQ ID NO: 234
  misc_feature 1..41: note = SYNTHETIC RNA
  source 1..41: mol_type = other RNA

SEQ ID NO: 274 - RNA, 41 nt, synthetic construct; identical to SEQ ID NO: 234
  misc_feature 1..41: note = SYNTHETIC RNA
  source 1..41: mol_type = other RNA

SEQ ID NO: 275 - RNA, 41 nt, synthetic construct; identical to SEQ ID NO: 234
  misc_feature 1..41: note = SYNTHETIC RNA
  source 1..41: mol_type = other RNA

SEQ ID NO: 276 - RNA, 44 nt, synthetic construct; identical to SEQ ID NO: 41
  misc_feature 1..44: note = SYNTHETIC RNA
  source 1..44: mol_type = other RNA

SEQ ID NO: 277 - RNA, 44 nt, synthetic construct; identical to SEQ ID NO: 41
  misc_feature 1..44: note = SYNTHETIC RNA
  source 1..44: mol_type = other RNA

SEQ ID NO: 278 - RNA, 44 nt, synthetic construct; identical to SEQ ID NO: 41
  misc_feature 1..44: note = SYNTHETIC RNA
  source 1..44: mol_type = other RNA

SEQ ID NO: 279 - RNA, 41 nt, synthetic construct; identical to SEQ ID NO: 77
  misc_feature 1..41: note = SYNTHETIC RNA
  source 1..41: mol_type = other RNA

SEQ ID NO: 280 - RNA, 41 nt, synthetic construct; identical to SEQ ID NO: 77
  misc_feature 1..41: note = SYNTHETIC RNA
  source 1..41: mol_type = other RNA

SEQ ID NO: 281 - RNA, 41 nt, synthetic construct; identical to SEQ ID NO: 77
  misc_feature 1..41: note = SYNTHETIC RNA
  source 1..41: mol_type = other RNA

SEQ ID NO: 282 - RNA, 44 nt, synthetic construct; identical to SEQ ID NO: 189
  misc_feature 1..44: note = SYNTHETIC RNA
  source 1..44: mol_type = other RNA

SEQ ID NO: 283 - RNA, 44 nt, synthetic construct; identical to SEQ ID NO: 189
  misc_feature 1..44: note = SYNTHETIC RNA
  source 1..44: mol_type = other RNA

SEQ ID NO: 284 - RNA, 44 nt, synthetic construct; identical to SEQ ID NO: 189
  misc_feature 1..44: note = SYNTHETIC RNA
  source 1..44: mol_type = other RNA

SEQ ID NO: 285 - RNA, 41 nt, synthetic construct; identical to SEQ ID NO: 234
  misc_feature 1..41: note = SYNTHETIC RNA
  source 1..41: mol_type = other RNA

SEQ ID NO: 286 - RNA, 41 nt, synthetic construct; identical to SEQ ID NO: 234
  misc_feature 1..41: note = SYNTHETIC RNA
  source 1..41: mol_type = other RNA

SEQ ID NO: 287 - RNA, 41 nt, synthetic construct; identical to SEQ ID NO: 234
  misc_feature 1..41: note = SYNTHETIC RNA
  source 1..41: mol_type = other RNA

SEQ ID NO: 288 - RNA, 41 nt, synthetic construct; identical to SEQ ID NO: 234
  misc_feature 1..41: note = SYNTHETIC RNA
  source 1..41: mol_type = other RNA

SEQ ID NO: 289 - RNA, 41 nt, synthetic construct; identical to SEQ ID NO: 234
  misc_feature 1..41: note = SYNTHETIC RNA
  source 1..41: mol_type = other RNA

SEQ ID NO: 290 - RNA, 41 nt, synthetic construct; identical to SEQ ID NO: 234
  misc_feature 1..41: note = SYNTHETIC RNA
  source 1..41: mol_type = other RNA

SEQ ID NO: 291 - RNA, 41 nt, synthetic construct; identical to SEQ ID NO: 234
  misc_feature 1..41: note = SYNTHETIC RNA
  source 1..41: mol_type = other RNA

SEQ ID NO: 292 - RNA, 41 nt, synthetic construct; identical to SEQ ID NO: 234
  misc_feature 1..41: note = SYNTHETIC RNA
  source 1..41: mol_type = other RNA

SEQ ID NO: 293 - RNA, 41 nt, synthetic construct; identical to SEQ ID NO: 234
  misc_feature 1..41: note = SYNTHETIC RNA
  source 1..41: mol_type = other RNA

SEQ ID NO: 294 - RNA, 41 nt, synthetic construct; identical to SEQ ID NO: 234
  misc_feature 1..41: note = SYNTHETIC RNA
  source 1..41: mol_type = other RNA

SEQ ID NO: 295 - RNA, 41 nt, synthetic construct; identical to SEQ ID NO: 234
  misc_feature 1..41: note = SYNTHETIC RNA
  source 1..41: mol_type = other RNA

SEQ ID NO: 296 - RNA, 41 nt, synthetic construct; identical to SEQ ID NO: 234
  misc_feature 1..41: note = SYNTHETIC RNA
  source 1..41: mol_type = other RNA

SEQ ID NO: 297 - RNA, 41 nt, synthetic construct; identical to SEQ ID NO: 234
  misc_feature 1..41: note = SYNTHETIC RNA
  source 1..41: mol_type = other RNA

SEQ ID NO: 298 - RNA, 41 nt, synthetic construct; identical to SEQ ID NO: 234
  misc_feature 1..41: note = SYNTHETIC RNA
  source 1..41: mol_type = other RNA

SEQ ID NO: 299 - RNA, 41 nt, synthetic construct; identical to SEQ ID NO: 234
  misc_feature 1..41: note = SYNTHETIC RNA
  source 1..41: mol_type = other RNA

SEQ ID NO: 300 - RNA, 41 nt, synthetic construct; identical to SEQ ID NO: 234
  misc_feature 1..41: note = SYNTHETIC RNA
  source 1..41: mol_type = other RNA

SEQ ID NO: 301 - RNA, 41 nt, synthetic construct; identical to SEQ ID NO: 234
  misc_feature 1..41: note = SYNTHETIC RNA
  source 1..41: mol_type = other RNA

SEQ ID NO: 302 - RNA, 41 nt, synthetic construct; identical to SEQ ID NO: 234
  misc_feature 1..41: note = SYNTHETIC RNA
  source 1..41: mol_type = other RNA

SEQ ID NO: 303 - RNA, 41 nt, synthetic construct; identical to SEQ ID NO: 234
  misc_feature 1..41: note = SYNTHETIC RNA
  source 1..41: mol_type = other RNA

SEQ ID NO: 304 - RNA, 41 nt, synthetic construct; identical to SEQ ID NO: 234
  misc_feature 1..41: note = SYNTHETIC RNA
  source 1..41: mol_type = other RNA

SEQ ID NO: 305 - RNA, 41 nt, synthetic construct; identical to SEQ ID NO: 234
  misc_feature 1..41: note = SYNTHETIC RNA
  source 1..41: mol_type = other RNA

SEQ ID NO: 306 - RNA, 41 nt, synthetic construct; identical to SEQ ID NO: 234
  misc_feature 1..41: note = SYNTHETIC RNA
  source 1..41: mol_type = other RNA

SEQ ID NO: 307 - RNA, 41 nt, synthetic construct; identical to SEQ ID NO: 234
  misc_feature 1..41: note = SYNTHETIC RNA
  source 1..41: mol_type = other RNA

SEQ ID NO: 308 - RNA, 41 nt, synthetic construct; identical to SEQ ID NO: 234
  misc_feature 1..41: note = SYNTHETIC RNA
  source 1..41: mol_type = other RNA

SEQ ID NO: 309 - RNA, 41 nt, synthetic construct; identical to SEQ ID NO: 234
  misc_feature 1..41: note = SYNTHETIC RNA
  source 1..41: mol_type = other RNA

SEQ ID NO: 310 - RNA, 41 nt, synthetic construct; identical to SEQ ID NO: 234
  misc_feature 1..41: note = SYNTHETIC RNA
  source 1..41: mol_type = other RNA

SEQ ID NO: 311 - RNA, 41 nt, synthetic construct; identical to SEQ ID NO: 234
  misc_feature 1..41: note = SYNTHETIC RNA
  source 1..41: mol_type = other RNA

SEQ ID NO: 312 - RNA, 41 nt, synthetic construct; identical to SEQ ID NO: 234
  misc_feature 1..41: note = SYNTHETIC RNA
  source 1..41: mol_type = other RNA

SEQ ID NO: 313 - RNA, 41 nt, synthetic construct; identical to SEQ ID NO: 234
  misc_feature 1..41: note = SYNTHETIC RNA
  source 1..41: mol_type = other RNA

SEQ ID NO: 314 - RNA, 41 nt, synthetic construct; identical to SEQ ID NO: 234
  misc_feature 1..41: note = SYNTHETIC RNA
  source 1..41: mol_type = other RNA

SEQ ID NO: 315 - RNA, 41 nt, synthetic construct; identical to SEQ ID NO: 234
  misc_feature 1..41: note = SYNTHETIC RNA
  source 1..41: mol_type = other RNA

SEQ ID NO: 316 - RNA, 41 nt, synthetic construct; identical to SEQ ID NO: 234
  misc_feature 1..41: note = SYNTHETIC RNA
  source 1..41: mol_type = other RNA

SEQ ID NO: 317 - RNA, 41 nt, synthetic construct; identical to SEQ ID NO: 234
  misc_feature 1..41: note = SYNTHETIC RNA
  source 1..41: mol_type = other RNA

SEQ ID NO: 318 - RNA, 41 nt, synthetic construct; identical to SEQ ID NO: 234
  misc_feature 1..41: note = SYNTHETIC RNA
  source 1..41: mol_type = other RNA

SEQ ID NO: 319 - RNA, 41 nt, synthetic construct; identical to SEQ ID NO: 234
  misc_feature 1..41: note = SYNTHETIC RNA
  source 1..41: mol_type = other RNA

SEQ ID NO: 320 - RNA, 41 nt, synthetic construct; identical to SEQ ID NO: 234
  misc_feature 1..41: note = SYNTHETIC RNA
  source 1..41: mol_type = other RNA

SEQ ID NO: 321 - RNA, 41 nt, synthetic construct; identical to SEQ ID NO: 234
  misc_feature 1..41: note = SYNTHETIC RNA
  source 1..41: mol_type = other RNA

SEQ ID NO: 322 - RNA, 41 nt, synthetic construct; identical to SEQ ID NO: 234
  misc_feature 1..41: note = SYNTHETIC RNA
  source 1..41: mol_type = other RNA

SEQ ID NO: 323 - RNA, 41 nt, synthetic construct; identical to SEQ ID NO: 234
  misc_feature 1..41: note = SYNTHETIC RNA
  source 1..41: mol_type = other RNA

SEQ ID NO: 324 - RNA, 41 nt, synthetic construct; identical to SEQ ID NO: 234
  misc_feature 1..41: note = SYNTHETIC RNA
  source 1..41: mol_type = other RNA

SEQ ID NO: 325 - RNA, 41 nt, synthetic construct; identical to SEQ ID NO: 234
  misc_feature 1..41: note = SYNTHETIC RNA
  source 1..41: mol_type = other RNA

SEQ ID NO: 326 - RNA, 41 nt, synthetic construct; identical to SEQ ID NO: 234
  misc_feature 1..41: note = SYNTHETIC RNA
  source 1..41: mol_type = other RNA

SEQ ID NO: 327 - RNA, 41 nt, synthetic construct; identical to SEQ ID NO: 234
  misc_feature 1..41: note = SYNTHETIC RNA
  source 1..41: mol_type = other RNA

SEQ ID NO: 328 - RNA, 41 nt, synthetic construct; identical to SEQ ID NO: 234
  misc_feature 1..41: note = SYNTHETIC RNA
  source 1..41: mol_type = other RNA

SEQ ID NO: 329 - DNA, 41 bp, synthetic construct
  source 1..41: mol_type = other DNA
taatttctactcttgtagatggaaagagaattgttttctcc

SEQ ID NO: 330 - RNA, 41 nt, synthetic construct; identical to SEQ ID NO: 234
  misc_feature 1..41: note = SYNTHETIC RNA
  source 1..41: mol_type = other RNA

SEQ ID NO: 331 - RNA, 41 nt, synthetic construct; identical to SEQ ID NO: 234
  misc_feature 1..41: note = SYNTHETIC RNA
  source 1..41: mol_type = other RNA

SEQ ID NO: 332 - RNA, 41 nt, synthetic construct; identical to SEQ ID NO: 234
  misc_feature 1..41: note = SYNTHETIC RNA
  source 1..41: mol_type = other RNA

SEQ ID NO: 333 - RNA, 41 nt, synthetic construct; identical to SEQ ID NO: 234
  misc_feature 1..41: note = SYNTHETIC RNA
  source 1..41: mol_type = other RNA

SEQ ID NO: 334 - RNA, 41 nt, synthetic construct; identical to SEQ ID NO: 234
  misc_feature 1..41: note = SYNTHETIC RNA
  source 1..41: mol_type = other RNA

SEQ ID NO: 335 - RNA, 41 nt, synthetic construct; identical to SEQ ID NO: 234
  misc_feature 1..41: note = SYNTHETIC RNA
  source 1..41: mol_type = other RNA

SEQ ID NO: 336 - RNA, 41 nt, synthetic construct; identical to SEQ ID NO: 234
  misc_feature 1..41: note = SYNTHETIC RNA
  source 1..41: mol_type = other RNA

SEQ ID NO: 337 - RNA, 41 nt, synthetic construct; identical to SEQ ID NO: 234
  misc_feature 1..41: note = SYNTHETIC RNA
  source 1..41: mol_type = other RNA

SEQ ID NO: 338 - RNA, 41 nt, synthetic construct
  misc_feature 1..41: note = SYNTHETIC RNA
  source 1..41: mol_type = other RNA
taatttctactcttgtagatcttgggtgtgttaaaagtgac

SEQ ID NO: 339 - RNA, 41 nt, synthetic construct; identical to SEQ ID NO: 338
  misc_feature 1..41: note = SYNTHETIC RNA
  source 1..41: mol_type = other RNA

SEQ ID NO: 340 - RNA, 41 nt, synthetic construct; identical to SEQ ID NO: 338
  misc_feature 1..41: note = SYNTHETIC RNA
  source 1..41: mol_type = other RNA

SEQ ID NO: 341 - RNA, 41 nt, synthetic construct; identical to SEQ ID NO: 338
  misc_feature 1..41: note = SYNTHETIC RNA
  source 1..41: mol_type = other RNA

SEQ ID NO: 342 - RNA, 41 nt, synthetic construct; identical to SEQ ID NO: 338
  misc_feature 1..41: note = SYNTHETIC RNA
  source 1..41: mol_type = other RNA

SEQ ID NO: 343 - RNA, 41 nt, synthetic construct
  misc_feature 1..41: note = SYNTHETIC RNA
  source 1..41: mol_type = other RNA
taatttctactcttgtagatacataaaactcttttaggtta

SEQ ID NO: 344 - RNA, 41 nt, synthetic construct; identical to SEQ ID NO: 343
  misc_feature 1..41: note = SYNTHETIC RNA
  source 1..41: mol_type = other RNA

SEQ ID NO: 345 - RNA, 41 nt, synthetic construct; identical to SEQ ID NO: 343
  misc_feature 1..41: note = SYNTHETIC RNA
  source 1..41: mol_type = other RNA

SEQ ID NO: 346 - RNA, 41 nt, synthetic construct; identical to SEQ ID NO: 343
  misc_feature 1..41: note = SYNTHETIC RNA
  source 1..41: mol_type = other RNA

SEQ ID NO: 347 - RNA, 41 nt, synthetic construct; identical to SEQ ID NO: 343
  misc_feature 1..41: note = SYNTHETIC RNA
  source 1..41: mol_type = other RNA

SEQ ID NO: 348 - RNA, 41 nt, synthetic construct; identical to SEQ ID NO: 343
  misc_feature 1..41: note = SYNTHETIC RNA
  source 1..41: mol_type = other RNA

SEQ ID NO: 349 - RNA, 41 nt, synthetic construct; identical to SEQ ID NO: 343
  misc_feature 1..41: note = SYNTHETIC RNA
  source 1..41: mol_type = other RNA

SEQ ID NO: 350 - RNA, 41 nt, synthetic construct; identical to SEQ ID NO: 343
  misc_feature 1..41: note = SYNTHETIC RNA
  source 1..41: mol_type = other RNA

SEQ ID NO: 351 - RNA, 41 nt, synthetic construct; identical to SEQ ID NO: 343
  misc_feature 1..41: note = SYNTHETIC RNA
  source 1..41: mol_type = other RNA

SEQ ID NO: 352 - RNA, 41 nt, synthetic construct; identical to SEQ ID NO: 343
  misc_feature 1..41: note = SYNTHETIC RNA
  source 1..41: mol_type = other RNA

SEQ ID NO: 353 - RNA, 41 nt, synthetic construct; identical to SEQ ID NO: 343
  misc_feature 1..41: note = SYNTHETIC RNA
  source 1..41: mol_type = other RNA

SEQ ID NO: 354 - RNA, 41 nt, synthetic construct; identical to SEQ ID NO: 343
  misc_feature 1..41: note = SYNTHETIC RNA
  source 1..41: mol_type = other RNA

SEQ ID NO: 355 - RNA, 41 nt, synthetic construct; identical to SEQ ID NO: 343
  misc_feature 1..41: note = SYNTHETIC RNA
  source 1..41: mol_type = other RNA

SEQ ID NO: 356 - RNA, 41 nt, synthetic construct; identical to SEQ ID NO: 343
  misc_feature 1..41: note = SYNTHETIC RNA
  source 1..41: mol_type = other RNA

SEQ ID NO: 357 - RNA, 41 nt, synthetic construct
  misc_feature 1..41: note = SYNTHETIC RNA
  source 1..41: mol_type = other RNA
taatttctactcttgtagatatagtctttccttgggtgtgt

SEQ ID NO: 358 - RNA, 42 nt, synthetic construct
  misc_feature 1..42: note = SYNTHETIC RNA
  source 1..42: mol_type = other RNA
taatttctactaagtgtagatatagtctttccttgggtgtgt

SEQ ID NO: 359 - RNA, 44 nt, synthetic construct
  misc_feature 1..44: note = SYNTHETIC RNA
  source 1..44: mol_type = other RNA
taatttctactaagtgtagatatagtctttccttgggtgtgtta

SEQ ID NO: 360 - RNA, 41 nt, synthetic construct; identical to SEQ ID NO: 338
  misc_feature 1..41: note = SYNTHETIC RNA
  source 1..41: mol_type = other RNA

SEQ ID NO: 361 - RNA, 42 nt, synthetic construct
  misc_feature 1..42: note = SYNTHETIC RNA
  source 1..42: mol_type = other RNA
taatttctactaagtgtagatcttgggtgtgttaaaagtgac

SEQ ID NO: 362 - RNA, 44 nt, synthetic construct
  misc_feature 1..44: note = SYNTHETIC RNA
  source 1..44: mol_type = other RNA
taatttctactaagtgtagatcttgggtgtgttaaaagtgacca

SEQ ID NO: 363 - RNA, 44 nt, synthetic construct; identical to SEQ ID NO: 362
  misc_feature 1..44: note = SYNTHETIC RNA
  source 1..44: mol_type = other RNA

SEQ ID NO: 364 - RNA, 42 nt, synthetic construct
  misc_feature 1..42: note = SYNTHETIC RNA
  source 1..42: mol_type = other RNA
taatttctactaagtgtagatacacacccaaggaaagactat

SEQ ID NO: 365 - RNA, 44 nt, synthetic construct
  misc_feature 1..44: note = SYNTHETIC RNA
  source 1..44: mol_type = other RNA
taatttctactaagtgtagatacacacccaaggaaagactatga

SEQ ID NO: 366 - RNA, 41 nt, synthetic construct
  misc_feature 1..41: note = SYNTHETIC RNA
  source 1..41: mol_type = other RNA
taatttctactcttgtagatatccgtgctgagtgtaccatg

SEQ ID NO: 367 - RNA, 42 nt, synthetic construct
  misc_feature 1..42: note = SYNTHETIC RNA
  source 1..42: mol_type = other RNA
taatttctactaagtgtagatatccgtgctgagtgtaccatg

SEQ ID NO: 368 - RNA, 44 nt, synthetic construct
  misc_feature 1..44: note = SYNTHETIC RNA
  source 1..44: mol_type = other RNA
taatttctactaagtgtagatatccgtgctgagtgtaccatgca

SEQ ID NO: 369 - RNA, 41 nt, synthetic construct; identical to SEQ ID NO: 61
  misc_feature 1..41: note = SYNTHETIC RNA
  source 1..41: mol_type = other RNA

SEQ ID NO: 370 - RNA, 42 nt, synthetic construct
  misc_feature 1..42: note = SYNTHETIC RNA
  source 1..42: mol_type = other RNA
taatttctactaagtgtagattaaacactgtttcatttcatc

SEQ ID NO: 371 - RNA, 44 nt, synthetic construct
  misc_feature 1..44: note = SYNTHETIC RNA
  source 1..44: mol_type = other RNA
taatttctactaagtgtagattaaacactgtttcatttcatccg

SEQ ID NO: 372 - RNA, 41 nt, synthetic construct
  misc_feature 1..41: note = SYNTHETIC RNA
  source 1..41: mol_type = other RNA
taatttctactcttgtagatgaaacgtcagtcttctctttt

SEQ ID NO: 373 - RNA, 42 nt, synthetic construct
  misc_feature 1..42: note = SYNTHETIC RNA
  source 1..42: mol_type = other RNA
taatttctactaagtgtagatgaaacgtcagtcttctctttt

SEQ ID NO: 374 - RNA, 44 nt, synthetic construct
  misc_feature 1..44: note = SYNTHETIC RNA
  source 1..44: mol_type = other RNA
taatttctactaagtgtagatgaaacgtcagtcttctcttttgt

SEQ ID NO: 375 - RNA, 41 nt, synthetic construct
  misc_feature 1..41: note = SYNTHETIC RNA
  source 1..41: mol_type = other RNA
taatttctactcttgtagattaatgccctgtagtctctctg

SEQ ID NO: 376 - RNA, 42 nt, synthetic construct
  misc_feature 1..42: note = SYNTHETIC RNA
  source 1..42: mol_type = other RNA
taatttctactaagtgtagattaatgccctgtagtctctctg

SEQ ID NO: 377 - RNA, 44 nt, synthetic construct
  misc_feature 1..44: note = SYNTHETIC RNA
  source 1..44: mol_type = other RNA
taatttctactaagtgtagattaatgccctgtagtctctctgta

SEQ ID NO: 378 - RNA, 41 nt, synthetic construct
  misc_feature 1..41: note = SYNTHETIC RNA
  source 1..41: mol_type = other RNA
taatttctactcttgtagattaattaacagcttgctggtga

SEQ ID NO: 379 - RNA, 42 nt, synthetic construct
  misc_feature 1..42: note = SYNTHETIC RNA
  source 1..42: mol_type = other RNA
taatttctactaagtgtagattaattaacagcttgctggtga

SEQ ID NO: 380 - RNA, 44 nt, synthetic construct
  misc_feature 1..44: note = SYNTHETIC RNA
  source 1..44: mol_type = other RNA
taatttctactaagtgtagattaattaacagcttgctggtgaaa

SEQ ID NO: 381 - RNA, 41 nt, synthetic construct; identical to SEQ ID NO: 73
  misc_feature 1..41: note = SYNTHETIC RNA
  source 1..41: mol_type = other RNA

SEQ ID NO: 382 - RNA, 42 nt, synthetic construct
  misc_feature 1..42: note = SYNTHETIC RNA
  source 1..42: mol_type = other RNA
taatttctactaagtgtagatggttaaagatggttaaatgat

SEQ ID NO: 383 - RNA, 44 nt, synthetic construct
  misc_feature 1..44: note = SYNTHETIC RNA
  source 1..44: mol_type = other RNA
taatttctactaagtgtagatggttaaagatggttaaatgattg

SEQ ID NO: 384 - RNA, 41 nt, synthetic construct; identical to SEQ ID NO: 77
  misc_feature 1..41: note = SYNTHETIC RNA
  source 1..41: mol_type = other RNA

SEQ ID NO: 385 - RNA, 42 nt, synthetic construct
  misc_feature 1..42: note = SYNTHETIC RNA
  source 1..42: mol_type = other RNA
taatttctactaagtgtagattgtgaaatggcttataattgc

SEQ ID NO: 386 - RNA, 44 nt, synthetic construct
  misc_feature 1..44: note = SYNTHETIC RNA
  source 1..44: mol_type = other RNA
taatttctactaagtgtagattgtgaaatggcttataattgctt

SEQ ID NO: 387 - RNA, 41 nt, synthetic construct
  misc_feature 1..41: note = SYNTHETIC RNA
  source 1..41: mol_type = other RNA
taatttctactcttgtagatgttgttggatttgaaattcca

SEQ ID NO: 388 - RNA, 42 nt, synthetic construct
  misc_feature 1..42: note = SYNTHETIC RNA
  source 1..42: mol_type = other RNA
taatttctactaagtgtagatgttgttggatttgaaattcca

SEQ ID NO: 389 - RNA, 44 nt, synthetic construct
  misc_feature 1..44: note = SYNTHETIC RNA
  source 1..44: mol_type = other RNA
taatttctactaagtgtagatgttgttggatttgaaattccaga

SEQ ID NO: 390 - RNA, 41 nt, synthetic construct
  misc_feature 1..41: note = SYNTHETIC RNA
  source 1..41: mol_type = other RNA
taatttctactcttgtagatttgtaggatatgcccttgact

SEQ ID NO: 391 - RNA, 42 nt, synthetic construct
  misc_feature 1..42: note = SYNTHETIC RNA
  source 1..42: mol_type = other RNA
taatttctactaagtgtagatttgtaggatatgcccttgact

SEQ ID NO: 392 - RNA, 42 nt, synthetic construct; identical to SEQ ID NO: 391
  misc_feature 1..42: note = SYNTHETIC RNA
  source 1..42: mol_type = other RNA

SEQ ID NO: 393 - RNA, 44 nt, synthetic construct
  misc_feature 1..44: note = SYNTHETIC RNA
  misc_feature 1: note = Terminal C3 spacer propanediol
  misc_structure 44: note = Terminal C3 spacer propanediol
  source 1..44: mol_type = other RNA
taatttctactaagtgtagatttgtaggatatgcccttgactat

SEQ ID NO: 394 - DNA, 27 bp, synthetic construct
  misc_feature 1..27: note = SYNTHETIC DNA
  source 1..27: mol_type = other DNA
aagaatgttgtgataaaaggtgatgct

SEQ ID NO: 395 - DNA, 24 bp, synthetic construct
  misc_feature 1..24: note = SYNTHETIC DNA
  source 1..24: mol_type = other DNA
acacatccatgggacttctgcctc

SEQ ID NO: 396 - DNA, 3834 bp, synthetic construct
  misc_feature 1..3834: note = SYNTHETIC DNA
  source 1..3834: mol_type = other DNA
atgctgaagaacgtgggcatcgaccggctggacgtggaaaagggcagaaagaacatgagcaagctcgagaagttcaccaactgctacagcctgagcaagaccctgcggttcaaggccattcctgtgggcaagacccaagagaacatcgacaacaagcggctgctggtggaagatgagaagagagccgaggactacaagggcgtgaagaagctgctggaccggtactacctgagcttcatcaacgacgtgctgcacagcatcaagctcaagaacctgaacaactacatcagcctgttccggaagaaaacccggaccgagaaagagaacaaagagctggaaaacctcgagatcaacctgcggaaagagatcgccaaggccttcaagggcaacgagggctacaagagcctgttcaagaaggacatcatcgagacaatcctgcctgagttcctggacgacaaggacgagatcgccctggtcaacagcttcaacggcttcacaaccgccttcaccggctttttcgacaaccgcgagaatatgttcagcgaggaagccaagagcacctctatcgccttccggtgcatcaacgagaatctgacccggtacatcagcaacatggatatcttcgagaaggtggacgccatcttcgacaagcacgaggtgcaagagatcaaagaaaagatcctgaacagcgactacgacgtcgaggacttcttcgagggcgagttcttcaacttcgtgctgacacaagagggcatcgatgtgtacaacgccatcatcggcggcttcgtgacagagagcggcgagaagatcaagggcctgaacgagtacatcaacctctacaaccagaaaacgaagcagaagctgcccaagttcaagcccctgtacaaacaggtgctgagcgacagagagagcctgtccttttacggcgagggctataccagcgacgaagaggtgctggaagtgttcagaaacaccctgaacaagaacagcgagatcttcagctccatcaagaagctcgaaaagctgtttaagaacttcgacgagtacagcagcgccggcatcttcgtgaagaatggccctgccatcagcaccatctccaaggacatcttcggcgagtggaacgtgatccgggacaagtggaacgccgagtacgacgacatccacctgaagaaaaaggccgtggtcaccgagaagtacgaggacgacagaagaaagagcttcaagaagatcggcagcttcagcctggaacagctgcaagagtacgccgacgccgatctgagcgtggtggaaaagctgaaagagattatcatccagaaggtcgacgagatctacaaggtgtacggcagcagcgagaagctgttcgacgccgactttgtgctggaaaagagcctcaaaaagaacgacgccgtggtggccatcatgaaggacctgctggatagcgtgaagtccttcgagaactatattaaggccttctttggcgagggcaaagagacaaaccgggacgagagcttctacggcgatttcgtgctggcctacgacatcctgctgaaagtggaccacatctacgacgccatccggaactacgtgacccagaagccttacagcaaggacaagtttaagctgtacttccagaatccgcagttcatgggcggctgggacaaagacaaagaaaccgactaccgggccaccatcctgagatacggctccaagtactatctggccattatggacaagaaatacgccaagtgcctgcagaagatcgataaggacgacgtgaacggcaactacgagaagattaactacaagctgctgcccggacctaacaagatgctgcctaaggtgttctttagcaagaaatggatggcctactacaaccccagcgaggatatccagaaaatctacaagaacggcaccttcaagaaaggcgacatgttcaacctgaacgactgccacaagctgatcgatttcttcaaggacagcatcagcagataccccaagtggtccaacgcctacgacttcaatttcagcgagacagagaagtataaggatatcgccgggttctaccgcgaggtggaagaacagggctataaggtgtcctttgagagcgccagcaagaaagaggtggacaagctggtcgaagagggcaagctgtacatgttccagatctataacaaggacttctccgacaagagccacggcacccctaacctgcacaccatgtactttaagctgctgttcgatgagaacaaccacggccagatcagactgtctggcggagccgagctgtttatgagaagggccagcctgaaaaaagaggaactggtcgttcaccccgccaactctccaatcgccaacaagaaccccgacaatcccaagaaaaccaccacactgagctacgacgtgtacaaggataagcggttctccgaggaccagtacgagctgcacatccctatcgccatcaacaagtgccccaagaatatcttcaagatcaacaccgaagtgcgggtgctgctgaagcacgacgacaacccttacgtgatcggcatcgacagaggcgagcggaacctgctgtatatcgtggtggtggacggcaagggcaatatcgtggaacagtactccctgaatgagatcatcaacaacttcaatggcatccggatcaagacggactaccacagcctgctggacaaaaaagagaaagaacgcttcgaggcccggcagaactggaccagcatcgagaacatcaaagaactgaaggccggctacatctcccaggtggtgcacaagatctgcgagctggttgagaagtatgacgccgtgattgccctggaagatctgaatagcggctttaagaacagccgcgtgaaggtcgagaaacaggtgtaccagaaattcgagaagatgctgatcgacaagctgaactacatggtcgacaagaagtctaacccctgcgccacaggcggagccctgaagggatatcagatcaccaacaagttcgagtccttcaagagcatgagcacccagaatggcttcatcttctacatccccgcctggctgaccagcaagatcgatcctagcaccggattcgtgaacctgctcaagaccaagtacaccagcattgccgacagcaagaagttcatctccagcttcgaccggattatgtacgtgcccgaagaggacctgttcgaattcgccctggattacaagaacttcagccggaccgatgccgactatatcaagaagtggaagctgtatagctacggcaaccgcatccgcatcttcagaaacccgaagaaaaacaacgtgttcgactgggaagaagtgtgcctgaccagcgcctacaaagaactcttcaacaaatacggcatcaactaccagcagggcgacatcagagccctgctgtgcgagcagagcgacaaggccttttacagctccttcatggccctgatgtccctgatgctgcagatgcggaatagcatcaccggcaggaccgacgtggacttcctgatcagccctgtgaagaattccgacgggatcttctacgacagcagaaactacgaggctcaagagaacgccatcctgcctaagaacgccgatgccaacggcgcctataatatcgccagaaaggtgctgtgggccatcggccagtttaagaaggccgaggacgagaaactggacaaagtgaagatcgccatctctaacaaagagtggctggaatacgcccagaccagcgtgaagcacggcagatctagtgacgatgaggccaccgccgatagccagcatgcagcccctccaaagaaaaagcggaaagtgctggaacaccaccaccatcaccac